European Patent Application EP 4 609 917 A2, published September 3, 2025. Title: Methods and Compositions for Treating Intestinal Disorder. Applicant: MARS, INCORPORATED. Application EP. The sequence listing filed with the application follows.

SEQUENCE LISTING (99 sequences)

SEQ ID NO: 1 - DNA, 11141 bp, Clostridium hiranonis
  source 1..11141: mol_type = genomic DNA
gcaaattgattttgattggtatttctttcattcaaaatatctcctttcctttatttagctgtattaaaatttataaaaaattttcattgttaataaaaaaatattctttgttagtattatagcataatttataaaaataatgataatgttttaatattgaaataataaatatgtaaaaaggttggaaatttatttaaaaatgaccagagataaaaagctcaggtcattttttttattattacaagtaatttgaaaaaaatatatgaaatgaatggagaaaatataactgagatacatttgataatgaaaaaaacatttatcgaaattgtaaatagactcattgttataattaataaatatttattatggcatagttgttaaaattataccctaaagaaacgtttcctcaaaaagtgggttataaaataaatgttttttgacgaaagatgtgattttatttgtaccccttttgtataaagattaaacagtatttttgtataaatatattgtatacagtatagagaatgtcgatgtaaaaaagtatataaaagtaaataataatcaaaaaaactagttttaattattaaaaatgataaaaaatattaataaaataaagagtcaaaaatacttgttagttaaatcacagattttgtctaagtatagattaggttttgtatttgaaaaggtcatctatagtgttgtaagaaagcgagttattagcacatattgtatctcaaaaaaatgttaagataatatcaagatagggcgataaagaaaaaagcaaattgaaaaagaaaaaagtaactataagtttttacaataaatcaaaagagaattgattttaaaagagggaggcaaaataccgatatgaatgatgtgaaatgtaaatattttaataaatttaatacaggaatgtcagattttgttactccaggaaaacagttagaatatgtagcaaaatgcaagccagatgaaaaagctatcatatatatagataaagaagacaatgtgagagatatcacttggaaggaacttcacatagcttcaaataaactagcttggcatttaatgaaaaagggatttggaaaaggtcaggtagcaatggtatctttcccaaatggtatagaacatatattagcaacattagctgtttggaaaacaggaggttgctacatgccagtttcttgtaagataacagatacagagcttggtgatatatgcagaataataaaaccaacagtttcttttacagataaagaaatgccttgtagaacagaaagtataaaaataggatcagtattcgatgtttgtaaagacgaatcagaagaaatgccagaagatatagctgcaaatccaaatatgatttctccatctggaggaacaacaggagagcctaagttcataaaacagaatgtggcaagtggcttatctgatgaaattataaaaagctggtttgaaatgtcaggtatggaatttgaacaaagacaattattagtaggaccacttttccatggtgctcctcatacagcagcatttaatggattatttgtaggaaatacattgataatacctagaaatttaagacctgaaagtatagttagatatataaaagaatacaaaatagaatttatacagatgatcccaacattaatgaatagaataataaaattagctgatgttgataaagaagattttaaatcaataaaagcactacaccatactggtggatattgttctccatatttaaaagaaaagtggatcgatataataggagctgaaaaagttcacgaaatgtactctatgacagaggcaatcggtatcacttgtataagaggagatgaatggcttaaacactatggaagcgtaggacttccactaggaggaagcagaatatcaataagagatgaagaaggaaatgaattaggaccacatgaggttggagaaattcatatgacttcaccaagtgcttgttgcatgacagaatacataaaccataaaccacttgaaactaaagatggtggatttagaagtgttggtgatttcggttatgtagatgaagatggatacctttacttctcagatagaagaagcgacatgcttgttataggtggagaaaacgtatttgcgactgaagttgaaccagtactaccagcttatgaaaaagtagttgatgctgtggtagttggaatacctgatgaagagtggggaagaagattacacgcaatagtacagaagaaagaagaagtttcagcagaagaattaatcgagtacttaggaaaacacttattaccatataaagttccaaagagctttacatttgttccttgcataccaagaggtgacaatggaaaggtaaacagagataagatgctaaaaggcttaatagaaaaaaatctagttaataaagtttgctaggatataaattcagttaactatctgcaccaagtgcagtggaaaataaatcaaaattaataaaataaattaataaggtaaatttaggaggtctaaaatgagttacgacgcacttttttcaccatttaaaatcagaggattagaacttaaaaacagaatagttctaccaggtatgaatacaaaaatggcaaaaaataaacatgatttaagcgatgatatgatagcttaccatgttgcaagagcaaaagcaggttgtgcattaaatatatttgaatgtgttgcgctatgtccagcacctcatgcatatatgtacatgggattatacaatgacaatcatgtagctcagttaaaaaaattaacagatgctgttcacgaagttggcggtaaaatggctgttcagttatggcatggtggtttcagcccacagatgttctttgataaaacaaatacattagaaacaccagatactataacagttgaacgtattcatgaaatagttaaagagtttggagaaggtgcaagaagagctgttgaagctggattcgatgcagttgaattccatgcagcacacagttacttacctcacgaattcctaagtccaggaatgaacaaaagaactgacgaatatggtggaaacttcgaaaatcgttgcagattctgcttcgaagtagttgaagctatacgtgcaaatataccagaagatatgccattcttcatgagagttgactgcatagatgagttaatggatgaagtaatgacagaagaagaaatagtagaattcataaatagatgtgctgatctaggagtagacgtagctgacttatcaagaggtaatgctcagtcattcgcaacagtttacgaagttcctcctttcaacttacagcacggtttcaatatagaaaacatatacaacatcaaaaaacagataaaaataccagtaatgggtgttggacgtataaacacaggagaaatggctaaccaggtaatagcagatggaaaatttgacttagttggtataggtcgtgctcagttagcagatcaggattgggttgctaaagttagagaaggtaaagaagatttaatacgtcattgtataggatgtgaccagggatgctacgatgcagttataaaccctcagatgactcatataacttgtacaagaaaccctcacttatgcttagaatacaaaggtatgccaaaaactgatgaacctaaaaaagttatgataatcggtggtggtatggctggtatattagcagctgaagtacttaaaaaacgtggacatgaaccagttatattcgaagcttctgatcacttagcaggacagttcgtattagcaggtaaagctccaatgaaagaagactgggcagctgcagctaaatgggaagctgaagaagtagctcgtttaggaatagaagttagatacaatacaaaagttactccagaattaatagaagaattcgctccagaccacgttgttatagctataggatctgattacgtagctccagctataccaggtatagatagtgacaaagtttacactcagtatcaggtattaaaaggtgaagtagaaccaaaaggacatgtagcagtagttggttgtggattagttggtacagaagttgctcagtacttagcagctagaggagctcaggtaacagctatagaaagaaaaggtgttggtacaggtctaagcatgcttagaagaatgttcatgaacccagaattcaaatactacaaaataaacaaaatgtctggaactaacatagttggtatagaaccaggaaaacttcactacataatgactaacaagaaaactcaggaagttactgaaggtgtgttagaatgtgatgcagcagtaatctgtacaggtataactgctagaccaagtgaagatttacaggaaaaatgtaaagaattaggtgttccattcaacgtaataggtgacgcagctggtgctagagatgctagaatagctactcaggaaggttacgaagtaggtatgagtatataatttaaaaattatataattatataaattaaaagttattaaattacaagaaagaggcgaataaaatgactttagaagcaagaatagaagcattagaaaaagaaatacagagattaaacgatatagaagctataaaacagttaaaagctaaatatttccgttgcctagatggaaaattatgggatgaattagaaactactctttctcctaacatagaaacttcttactctgatggaaaattagtattccacagcccaaaagaagtaactgaatatttagcagcagcaatgcctaaagaagaaataagtatgcacatgggacatactccagaaataactatagacagcgaaaatactgctacaggaagatggtacttagaagataacctaatattcacagacggaaaatacaaaaacgttggaataaacggtggagcattctacacagataaatatgaaaaaatagacggacagtggtacataaaagaaactggatatgttcgtatatttgaagaacatttcatgagagatccaaaaatacatataactagcaacatgcataaagaaaaataataactgattgctaataaacaagatataaacagggggctggtaaacagccagccctctgaaaaataaactaaaaaactataatcttttaaaatcttaattaaagtagaaggagataagacaatgaacttagtacaggacaaaatagttataataacaggtggaacaagtggtataggtctttgcgcagcaaaaatattcatggataacggtgcaacagtttctatattcggaaaaactcaggaagaagtagatgctgctaaagcagaattaaaagaaactcacccagataaagaagtattaggatttgctccagatttaactaatagagatgaagttatggctgcagttggtgcagtagctgaaaaatacggaagattagacgttatgataaacaatgctggtgttactagctcaaacgtattctcaagagttagcccagaagaattcacatatttaatggatataaacgttacaggtgtattccatggtgcttgggctgcttaccactgcctgaaaggtgaaaagaagattataataaatactgcttcagtaacaggaatacacggatcattatcaggagttggatacccaacaagtaaatcagctgttgtaggattcactcaggctcttggtagagaaataatacgtaaaaacataagagttgttggtgttgcaccaggtgttgttaacactccaatggttggtaatataccagatgaaatattagatggatacctaagctcattcccaatgaagagaatgttagaaccagaagaaatagctaacacttacttattcttagcttctgacttagctagtggtataacagctacaactgtaagcgttgacggtgcttatagaccatcataagatttactttaatttaaaactgtaattagatagataatacgacgattaatataaaaaatgttctttaaaagaaaaggagaaataaaatggctggattaaaagattttcctaaatttggtgcactttctggattaaaaatattagatagtggatctaacatagctggacctctaggtggtggacttttagcagaatgtggtgctacagttatacacttcgaaggacctaaaaaacctgacaaccagagaggttggtatggataccctcagaaccacagaaaccagttatcaatggttgctgatataaaatctgaagaaggtagaaaaatattcttagacttaataaaatgggctgacatatgggttgaatcatcaaaaggtggacagtacgacagactaagtctttctgatgaagttatatggtcagtaaaccctaaaatagctatagttcacgtttctggatacggacaggttggagatccatcatacgtaacaaaagcttcttatgatgctgttggacaggcattcagtggatacatgtcattaaatggtgttaatgaagcattaaaaataaatccttacctaagtgacttcgtatgtgttcttactacttgctgggcaatgttagcatgctacgtaagtactcagttaactggaaaaggagaatctgtagacgttgctcagtacgaagcattagctcgtataatggacggacgtatgatacagtacgctactgatggtgtaagtgttccaaaaactggtaacaaagatgctcaggcagctctattcagcttctatacttgtaaagatggaagaactatattcataggtatgactggtgctgaagtatgtaagagaggattccctgtaatagggcttccagttcctggtacaggtgaccctgacttcccagaaggattcacaggatggatgataaatactccagttggacagagaatggaaaaagctatggaagcattcgttgctgaaagaactatgccagaagttgaaaaagctatgatagatgctcagataccatgccagagagtttatgatcttgaagactgcttaaacgaccctcactggaatgctcgtggaactataatggaatgggatgacccaatgatgggacacataaaaggtcttggattaataaacaaattcaaaaacaacccttctgaaatatggagaggtgctccattattcggtatggacaacagagacataattagagaccttggatattctgaggaggaagttaacgatttatacgctaaaggtattgtaaacgaattcgaccttgaaacaactataaaacgttacaaacttgatcaggttatacctcacatggctaaaaaagataaataagaaacgtattaaataataaaatataaatgtcgagcctgccagaatgagaattttgacaggcttgatattataacgaaatgttataaaaaaaacaaaataaaaattgcttaaattttatacaaggagaattgaaatgacagcaacaaacgcaaactataaaaaaggctttatcccatttgctatagcagcgttactagtaggtcttataggtggtttcacagccgttctagcacctgcattcgtagcagatatgggtcttaacgataacaatactacatggatagcactagcgcttgcaatgtctacagctgcatgtgctccaatacttggtaaattaggtgacgtacttggacgtcgtaaaactttattattaggaatcatagtattcacaataggtaacgtattaacagcaatagcatcttcattaatattcatgctaggtgcaagatttatagttggggttggtacagcggctatagctccagttataatggcttacatagttacagaatatccaccagaagaaactggtaagggattcgctctttatatgttaatatcaagtgctgcagttgttgttggtccaacttgtggtggattaataatgcaggcatttggatggagaatgatgatgtgggtttgtgttgccctttgtgtagtaacattcttcatatgttcagtaatgattaagaaaacagactttgaaaagaaaagtcttgataacttcgataaaaaaggtgcagtatgcgtactaatattcttcagtttagtattatgtataccatcatttggacagaatataggttggacatcagcgccattcctaggtgttacagcagtagctttagtaacattattcttattaataaaagctgaaagcagtgcagaaaacccaatattaagtggtaaatttatgaaacgtaaagaattcatattaccagtattaatattattccttactcagggattaatgcaggctaacatgactaacgtaatattattcgttagagctactcagccagaaaatacaataatatcaagtttcgcaatatcaatcctttacataggtatgtctttaggttcagtattcataggacctatggcagataaaaaagaaccaaaaactgtacttacaggatcacttctattcactggtataggttgtgcaatgatgtacttcttcacagaaactgcaccattcgcaatgttagctggatctctaggaatgttaggtataggacttggaggaaatgctacaatactaatgaaagtttcattatctggattatctcaggcagaagctggatcaggaacaggaacatacggattattcagagatatatcagctccatttggtgttgcggtattcgtaccactatttgcaaacacagttacaacaagaatggctggagtaatggctaacggaactgcagaagctgctgctaaatcattagcatctgtttcttctatacatacattagcattagttgaagtatgctgtgtaatattagcaatagttgcagttagaatgctaccaaaaatacacaataaataatttaaaaataataacagagttgaaaaaacactcaattaaaagaggggccttgagccccttttttagtgtaaaaatgacaaaatactatcaatttatataaatgataattaaactcgtcaaccaaagaaatattcacaaagtagataataatagatattcaaaaagtgatatattattaggcaaaaagtgcaagaaattagcgagtattcgacaactttttgtccaatggtagaaaagaatatttgttatcataaatatagacaaagggctttgaccaaaactaaggaaaaagtttgcataatataaaaaataaaataaaataaaaaaataaaaataaaataaaagcgaaaggaaaaaacaacatcatggatatgaaaaattctaaactattctcacctttaacaataggatcattaacattaaacaacagagttggtatggcaccaatgagtatggactacgaagctgctgacggaacagttccaaaaagattagcagatatatttgttcgtagagctgaaggtggaacaggatatgtaacaatagacgcggtaacaatagatagtaaatataaatatatgggtaatacaactgctttagattctgatgatttagttactcagttcaaagaatttgcaacaagagttagagaagcaggaagcacattaatacctcaggttatacatccaggaccagaatcaatatgtggatacagacacatagcaccacttggaccatcagttaatacaaatgctaactgccacgtgagccgtgctataagtgtagatgaaatacatgaaataataaaacagtttggacaggctgctagaagagttgaagaagcaggatgcggtggtataggattacactgtgcacatgcttacatgctaccaggttcattcttatctccattaagaaacaaaagaatggatgaatacggcggatgtctagataacagagcaagattcgtaatagaaatgatagaagaagttcgtagaaatgtaagtcctgatttcccaataatgcttagaatatctggggatgaaagaatgataggaggaaactctttagaagatatgttatacttagctccaaaatttgttgaagctggtgtaaatatgtttgaagtttctggaggtactcagtacgaaggattagaacacataataccaagtcagaacaaaagcataggtgtaaacgtacacgaagcatctgaaatcaaaaaagttgtagatgttccagtttacgctgttggtaaaataaatgacataagatacgctgctgaaatagttgaaagaggactagttgatggggtatcaataggtagaccattattagcagatccagacttatgtaataaagcaaaagaaaacttatttgatgaaataactccatgtgcaagctgtggaggaagctgtataagccgtactgcagatagacctcagtgtcgttgccatataaacccaagagttggattcgaatatgattatccagaagttccagctgaaaaatctaaaaaagttctagttgtaggtgctggacctggtggtatgatggcagcagttacagcagctgaaagaggacatgatgtaacactttgggaagctgacactcagataggtggacagataaacttagcagtagtagctccaggtaaacaggaaatgactaaatggttatctcacttaaactacagagctaaaaaagctggagttaaaatggtattaggaaaagaagctacagtagaaaacataaaagaatttgctccagaagcagttatagttgcaacaggtgctagaccattagttccaccaataaaaggaactcaggactacccagttcttacagctcatgacttcttaagaggaaaattcgttataccaaaaggaaaagtttgtgtactaggtggaggagctgttgcttgtgaaactgcagaaacagtattagaaaacgctagaccaaacgcattcactagaggatttgatgctagtatcggtgatgtagatgttacattagtagaaatgttaccacagttattaacaggagtatgtgctccaaatagaactccattaataagaaaacttaaaaacaaaggtgttcatataaatgtaaatactaaaatattagaagtaactgaccacgacgttaaagttcagagagctgacggtgcagaagaatggttaaaaggattcgactacatactattcggacttggttctagaaactacgatccaatatctgaacagataaaagaattcgttccagaagtacacgttgttggggatgctaagagagctagacaggcaagctttgcaatgtgggaagctttcgaagcagcatacagcttataa

SEQ ID NO: 2 - DNA, 1393 bp, Clostridium hiranonis
  source 1..1393: mol_type = genomic DNA
acatgcaagtcgagcgattctcttcggagaagagcggcggacgggtgagtaacgcgtgggtaacctgccctgtacacacggataacataccgaaaggtatgctaatacgggataatatataagagtcgcatgacttttatatcaaagatttttcggtacaggatggacccgcgtctgattagcttgttggcggggtaacggcccaccaaggcgacgatcagtagccgacctgagagggtgatcggccacattggaactgagacacggtccaaactcctacgggaggcagcagtggggaatattgcacaatgggcgcaagcctgatgcagcaacgccgcgtgagcgatgaaggccttcgggtcgtaaagctctgtcctcaaggaagataatgacggtacttgaggaggaagccccggctaactacgtgccagcagccgcggtaatacgtagggggctagcgttatccggatttactgggcgtaaagggtgcgtaggcggtctttcaagtcaggagttaaaggctacggctcaaccgtagtaagctcctgatactgtctgacttgagtgcaggagaggaaagcggaattcccagtgtagcggtgaaatgcgtagatattgggaggaacaccagtagcgaaggcggctttctggactgtaactgacgctgaggcacgaaagcgtggggagcaaacaggattagataccctggtagtccacgctgtaaacgatgagtactagttgtcggaggttaccccttcggtgccgcagctaacgcattaagtactccgcctggggagtacgcacgcaagtgtgaaactcaaaggaattgacggggacccgcacaagtagcggagcatgtggtttaattcgaagcaacgcgaagaaccttacctaggcttgacatccttctgaccgaggactaatctcctctttccctccggggacagaagtgacaggtggtgcatggttgtcgtcagctcgtgtcgtgagatgttgggttaagtcccgcaacgagcgcaacccttgtctttagttgccatcattaagttgggcactctagagagactgccagggataacctggaggaaggtggggatgacgtcaaatcatcatgccccttatgcctagggctacacacgtgctacaatgggtggtacagagggcagccaagccgtgaggtggagcaaatcccttaaagccattctcagttcggattgtaggctgaaactcgcctacatgaagctggagttactagtaatcgcagatcagaatgctgcggtgaatgcgttcccgggtcttgtacacaccgcccgtcacaccatgggagttggagacacccgaagccgactatctaaccttttgggagaagtcgtccccctcgaatcaatacccc

SEQ ID NO: 3 - DNA, 9743 bp, Clostridium scindens
  source 1..9743: mol_type = genomic DNA
aaaagatattaagcattaagaaaatgcacaaaaaatcagcgtgtgagagggagggcaaggagttgaagcgtgacttttttaacaagtttaatttggggacatcgaactttgtcacgccgggaaaacagttggaatacgtttcggaatgcaagccagattctactgcggtcatttgcttagataaagaacagaactgttccgttattacttggcatcagctgcacgtctattccagccagctggcatggtaccttatagaaaatgagattggcccggggtcgatcgtacttacaatgtttccgaacagcatcgagcacattattgcggtatttgcaatctggaaggcgggcgcctgctatatgcccatgtcctataaggcggcggaatccgagatcagggaggcctgcgataccatccacccgaatgcggcttttgcggaatgcaagattccaggattaaaattctgccttagcgcagacgagatatatgaggcgatggaaggaagatccaaggagatgccttcggaccgtctggccaatccgaacatgatatccttatcaggcggaaccagcggaaagatgaagttcatccgtcagaaccttccatgcgggctggacgatgagacgatcagaagctggtctttgatgtctggaatgggatttgagcagcgccagctgctggtaggcccgctgtttcatggcgcgcctcactccgcggcgtttaatggactgttcatgggcaacaccctggtactgaccaggaacctttgcccgggaaatatcctgaacatgattaagaaatataagattgaatttatacagatggtgccgaccctgatgaaccggcttgccaaactggagggagtcggaaaagaagactttgcatccctgaaggcgctgtgccatacagggggcgtctgttctccctggcttaagcagatctggatcgacctgctggggcctgaaaagatctatgagatgtattccatgacggaatgcatcggccttacctgcatccggggagacgagtgggtgaagcatccgggaagcatcggacggccagtgggcgatagcaaggtgtctatccgggatgagaatggcaaggaagttgcgccttttgagattggcgagatctatatgacagcgccggcctcctatctggttaccgagtacatcaattgggaaccgctggaagtgaaagagggaggcttccgaagcgtaggggatatcggctacgtggatgagcagggctatctgtacttttctgaccggcgcagcgacatgctggtatcaggcggagaaaacgtgttcgccaccgaagtcgagacggcgcttttgagatataaggatatcctggacgctgtagtggtagggataccggatgaagatctggggcgaaggctccatgcggtcattgagacagggaaagagataccggcagaggaactgaaaacattcctgagaaagtatctgactccatataagataccaaagacgttcgagttcgtaaggagcatacgaaggggagacaatggaaaggccgacaggaagcggatcctggaagattgtattgcccgcgggggatgattctataaatgcaaagaaaacaaattatataaaggaggagtaacaaaatgagttacgaagcacttttttcaccattcaaggtcagaggactggaacttaaaaaccgtatcgtcctgcctggaatgaacaccaagatggcaaagaacaagcacgacataggcgaggatatgatagcctaccatgttgccagggcaaaagcgggatgcgcgttaaatatatttgaatgcgtagcattatgtccggcgcctcacgcttatatgtatatggggctttatacggaccatcatgtagaacagcttaagaaattgacggatgcagtccatgaagcaggcggcaagatgggcatccagctgtggcatggaggattcagcccgcagatgttctttgacgagaccaacaccctggaaactccggacactcttacggtagagaggattcatgagatcgtagaagaattcggacgcggcgcaaggatggctgttcaggctggatttgacgcagtagaattccatgcggctcacagttatctgcctcacgagttcttaagccctggaatgaacaaacgtacggatgagtacggcggaagttttgagaaccgctgcagattctgttatgaagtcgttcaggcaatccgttccaatatcccggatgacatgccattctttatgcgtgcagactgcatcgacgaattaatggaacagaccatgacagaggaagagatcgttacatttatcaataagtgcgcagaacttggcgtggatgtggcagacctttcccgtggaaacgcgacttcattcgcaaccgtatatgaagttccgccattcaacctggctcatggcttcaacatagagaatatttacaacatcaaaaagcagatcaatatcccggttatgggagttggccgtatcaatacaggagagatggcaaacaaggtcattgaagaaggcaagtttgacctggtaggcatcggacgcgcccagcttgcagatccaaactggatcaccaaagtaagagaaggcaaagaagacctgatccgccactgtatcggatgtgaccagggatgctatgacgcagtcatcaatccaaagatgaagcatatcacctgcacccacaatccaggattgtgcttagagtatcagggaatgccaaagacagacgctcctaagaaagtcatgatcgtaggaggcggaatggcaggcatgatcgctgcggaagtattaaagaccagaggccataacccggtaatcttcgaggcatccgacaagcttgcaggacagttcaggctggcaggcgtagcgccgatgaagcaggattgggcagatgttgcagaatgggaagcaaaagaagtagagcgccttggaatcgaagtacgtctgaataccgaagtgactgcagagaccatcaaggaattcaatccggataatgtcatcatcgcagtaggctctacctatgcgctgcctgagattccgggaatcgacagcccaagcgtatactcccagtatcaggtactgaaaggggaagtaaatccgacaggccgtgtagccgttatcggatgcggactggttggtacggaagtcgcagaacttctggcatccagaggcgcacaggtaatcgcgatcgagaggaagggcgtaggtaccggccttagcatgcttcgcagaatgttcatgaacccggaattcaaatattacaagatcgccaagatgtccggaacaaatgtcaccgctttagagcagggcaaggttcactacatcatgacagacaagaagaccaaagaagtgacgcagggagtcctggaatgcgacgctaccgttatctgtacaggaattaccgcacgtccaagcgatgggcttaaggcaagatgcgaagaacttggaatcccggttgaggtgatcggagacgctgctggcgcaagagactgcacgatcgcgacacgcgaaggctatgacgcaggaatggcaatctagaaaatcagaacttatcaatcttacatatagaaaggatgatacatatgacattagaagagagagttgaagcattagaaaaagaattgcaggagatgaaggatattgaggcaatcaaggaactgaaaggaaagtatttccgctgcctggacggaaagatgtgggatgagctggagaccaccctgtcaccaaatatcgtaacctcttattccaacgggaaactggtattccatagcccgaaggaagttaccgattacttaaagagctcgatgccaaaagaagagatcagcatgcatatgggccacacgccggagatcaccattgacagcgagactacggctacgggcagatggtatctggaagatagactgatctttacggacggtaagtacaaagacgtaggaatcaatggcggcgcgttctatacagacaaatatgagaagatagacggccagtggtacatccttgaaaccggctatgtacgaatctatgaagaacatttcatgcgtgatccaaagatccatatcacgatgaacatgcacaaataagaatattgtaaaagaaaggcaggagtaagagtatgaatctcgtacaagacaaagttacgatcatcacaggcggcacaagaggtattggattcgccgctgccaaaatatttatcgacaatggcgcaaaagtatccatcttcggagagacgcaggaagaagtagatacagcgcttgcacagttaaaagaactttatccggaagaagaggttctgggattcgcgccggatcttacatccagagacgcagttatggcagcggtaggccaggtagcacagaaatatggcagactggatgtcatgatcaacaatgcaggaattaccagcaacaacgtattctccagagtgtctgaagaagagttcaagcatattatggacatcaacgtaacaggcgtattcaacggcgcatggtgcgcataccagtgcatgaaggatgccaaaaagggcgttatcatcaacacggcatccgttacaggcatcttcggatcactctcaggcgtaggatatccggccagcaaggcaagcgtgatcggactcacccatggacttggaagagagatcatccgcaagaatatccgtgtagtaggagtggctcctggagttgtgaacacggatatgaccaatggcaatcctccggagatcatggaaggatatctgaaggcgcttccgatgaagagaatgcttgagccggaagagatcgctaatgtatacctgttcctggcatctgacttggcaagcggcattacggctactacggtcagcgtagacggggcttacagaccataattttaatttttactaagtagaatatgtgatatagaaaaggagatataaaaacatggctggaataaaagattttccaaaattcggagctcttgcagggcttaagatacttgacagcggatctaacatcgccggacctttaggcggaggccttctggcagaatgcggagcaacggtcatccattttgaaggaccaaagaaacctgataaccagagaggatggtacggctatccacagaatcaccgtaatcagctgtctatggtagcagacatcaaatctgaagaaggaagaaagatcttccttgatctgatcaaatgggcagatatctgggtagagtcatccaaaggcggacagtatgacaggctgggactttccgatgaagtcatctgggaagtaaatcctaagattgccatcgtgcacgtatccggatatggacagacaggagacccgtcttacgttacacgtgcatcctatgacgcagtaggccaggcattcagcggctatatgtcactgaacggaacaacggaagcgctgaagatcaatccttatctgagcgatttcgtatgcggacttaccacatgctgggctatgcttgcctgctatgtaagcaccattcttaccggaaaaggcgaatctgttgacgttgcacagtacgaagcgctggcacgtatcatggacggacgtatgatccagtacgctacagacggcgtgaagatgccaagaaccggcaataaggatgcgcaggctgccctgttcagcttctacacctgtaaagacggacgtacgatctttatcggaatgactggcgcggaagtatgtaagagaggcttcccgatcatcggacttccggtacctggaaccggagacccggacttcccggaaggcttcacaggctggatgatctatactcctgtaggacagagaatggaaaaggctatggagaagtatgtatctgagcatacgatggaagaagtagaggctgagatgcaggcacaccagattccatgccagagagtatacgagctggaagactgcctgaacgatcctcactggaaagcacgtggaactattacggagtgggatgacccgatgatgggacatatcacaggccttggactgatcaacaagttcaagagaaatccttccgaaatctggagaggcgctccgctgttcggtatggataaccgcgatatcctgaaagacctgggatatgacgatgcaaagatcgatgaactctatgagcagggcatcgtcaatgaattcgaccttgacactactatcaaacgctatagactggatgaagtaattccacatatgagaaagaaagaggagtaagagtatgagcaccgtagccaatccaaattataagaaaggttttgtcccctttgcaattgcagcactcctggtgagcctgatcggcggttttaccgccgttctcggcccggccttcgtggcggaccaggggattgactataataataccacatggatttccctggcgctggcgatgtcttccgccgcatgcgctccaatccttggaaaactgggagacgtgctaggacgcaggacgacgctgcttctgggtattgtgatctttgcggccggcaatgtgctgacagccgtagccacgtccctgatattcatgctggcagcccgttttatcgtaggtatcggaacagcagcgatctcaccgatcgttatggcctatatcgtaaccgagtatccgcaggaggagacaggaaaggcctttggcctgtatatgctgatctccagcggcgccgtcgtggtaggacctacctgtggcggcctgatcatgaatgcggctggctggagagtcatgatgtgggtatgcgtcgctctgtgcgtcgttgtattcctgatctgcacattctccatcaagaagactgcatttgagaagaagagcatggcaggatttgacaagccgggcgcagccctggtagtcgtattcttcagtttgttcctgtgcatcccatccttcggacagaatatcggatggtcttccacagcatttatcgcagcagcggcagtagcgctggtagcacttttcatcctggtaatggtagaaaagaaagcgaagagtccgatcatgaacggcaagtttatggcacgcaaggaattcgtgcttccagtattgatcctgttccttacacagggacttatgatggcaaatatgaccaatgtcatcgtgttcgtgcgctatacgcagccggacaatgtcattatatcaagttttgcgatctccatcatgtacataggaatgtccttaggctccgttatcattggacctgttgcagataagaaagagccaaagacggttctgacattctctctggtactgacagccatcggctgtgcgctgatgtatctgttcaaggcagattcctccgtcgctatctttgcggcatccttgggaatccttggatttggccttggaggaaatgcaaccatcttcatgaaggtagcgctttccggcctgtccagcgaagtagctggctctggtactggaacctatggcctgttcagagatatctcggcaccattcggcgtggcagtgttcgtgcctatgtttgccaacggcgtaacagcgaatattgcgaaatacgcgtcaggcggcatggaagaaggcgccgctacggtaaaagcagccatctcatccatccagacgctgacactggttgaacttggatgtatcgttgtgggaatcatccttgtgagaatgctgccaagaatctatcagaagaaagaggcataaataagttaagaaaagaggtaattataaatggatatgaaacattccagattattttcgccgcttcagatcggatccctgacactgtctaaccgtgtcggcatggctcccatgagcatggactatgaagcagcagacggaactgtgcccaagaggctggcggacgtatttgtccgccgcgccgagggaggcacaggctacgtcatgatcgacgcggtgacgatagacagcaagtatccttatatgggaaatacaacggcccttgaccgtgatgaactggttccccagtttaaggaatttgctgacagagtaaaagaagcaggcagcacgctggtgccgcagatcattcatccgggtccggaatccgtatgcggctaccggcatatcgctccgcttggaccttctgccaacaccaatgcaaactgccacgtgagcagatcgatcagcatagatgagatccatgacatcattaagcagttcggccaggcggcacgccgcgccgaagaagcaggatgcggggcaatctccctgcactgcgcgcatgcgtatatgctgccaggatccttcctgtcaccgcttcgcaacaagcgcatggatgaatatggcggaagccttgacaaccgtgcccgtttcgtgatcgagatgattgaggaggcccgcaggaatgtgagtcctgatttcccgatcttccttcgtatctccggagacgagagaatggtaggaggcaacagccttgaagatatgctctacctggcaccgaagttcgaggctgccggcgtaagcatgctggaagtatccggcggaacccagtatgaaggcctggaacatatcattccttgccagaataagagcaggggcgtcaatgtatatgaagcttctgagatcaagaaagtagtgggcatcccggtatacgcagtaggaaagatcaacgatatacgctatgcggcagagatcgtagaacgcggcctggtagacggcgtggctatgggacgtccgcttctggcagatccggacctttgcaagaaggcagtggaaggccagtttgacgagatcactccatgcgcaagctgcggcggaagctgcatcagccgttctgaggcagcgcctgagtgccattgccatattaatccaaggcttggccgggagtatgaattcccggatgtgcctgccgagaagtccaagaaggtactggttatcggcgcaggccctggaggaatgatggctgccgtgacagctgcggaacgcggccatgatgttacggtatgggaggctgacgacaagatcggcggccagctgaacctggcagtagtggctcctggcaagcaggagatgacccagtggatggtacatctgaactatcgcgcgaagaaagcaggcgtgaagtttgaattcaataaagaagcgacggcagaagatgtcaaggcgctggcgccggaagcagtgatcgttgctacaggcgcgaagccgctggttcctccgattaaaggaacacaggattatccggtgcttactgcccatgatttccttcgcggcaagttcgtgattccgaagggacgcgtctgcgtgctgggaggaggcgcggttgcctgcgagactgccgagacagccctggagaatgcacgtccgaattcttataccagaggatacgatgcaagcatcggagatatcgatgtcacgcttgtggagatgcttccgcagctccttaccggcgtatgcgcgccgaaccgcgagcctttgatccgcaagttaaagagcaagggcgtacacatcaacgtcaataccaagatcatggaagtaacagaccatgaagtaaaggttcagagacaggatggaacgcaggaatggctggaaggatttgactatgtcctctttggccttggttccagaaattacgatccgctttcagagaccctcaaggaattcgttccggaagtacatgtcatcggcgatgccgtaagggcgcgccaggcaagctacgcaatgtgggaaggatttgagaaggcatacagcctgtaaaagcggtttgagtaaaaggaggcttaagaaatggcagtgaaggcaatctcaggctgcgacaaggatcaggaactgatca

SEQ ID NO: 4 - DNA, 1531 bp, Clostridium scindens
  source 1..1531: mol_type = genomic DNA
gagagtttgatcctggctcaggatgaacgctggcggcgtgcctaacacatgcaagtcgaacgaagcgcttccgctagattttcttcggagatgaaggcggctgcgactgagtggcggacgggtgagtaacgcgtgggcaacctgccttgcactgggggataacagccagaaatggctgctaataccgcataagaccgaagcgccgcatggcgcagcggccaaagccccggcggtgcaagatgggcccgcgtctgattaggtagttggcggggtaacggcccaccaagccgacgatcagtagccgacctgagagggtgaccggccacattgggactgagacacggcccagactcctacgggaggcagcagtggggaatattgcacaatgggggaaaccctgatgcagcgacgccgcgtgaaggatgaagtatttcggtatgtaaacttctatcagcagggaagaagatgacggtacctgactaagaagccccggctaactacgtgccagcagccgcggtaatacgtagggggcaagcgttatccggatttactgggtgtaaagggagcgtagacggcgatgcaagccagatgtgaaagcccggggctcaaccccgggactgcatttggaactgcgtggctggagtgtcggagaggcaggcggaattcctagtgtagcggtgaaatgcgtagatattaggaggaacaccagtggcgaaggcggcctgctggacgatgactgacgttgaggctcgaaagcgtggggagcaaacaggattagataccctggtagtccacgccgtaaacgatgactactaggtgtcgggtggcaaggccattcggtgccgcagcaaacgcaataagtagtccacctggggagtacgttcgcaagaatgaaactcaaaggaattgacggggacccgcacaagcggtggagcatgtggtttaattcgaagcaacgcgaagaaccttacctgatcttgacatcccgatgccaaagcgcgtaacgcgctctttcttcggaacatcggtgacaggtggtgcatggttgtcgtcagctcgtgtcgtgaggtgttgggttaagtcccgcaacgagcgcaacccctatcttcagtagccagcatttcggatgggcactctggagagactgccagggacaacctggaggaaggtggggatgacgtcaaatcatcatgccccttatgaccagggctacacacgtgctacaatggcgtaaacaaagggaggcgaacccgcgagggtgggcaaatcccaaaaataacgtctcagttcggattgtagtctgcaactcgactacatgaagctggaatcgctagtaatcgcgaatcagaatgtcgcggtgaatacgttcccgggtcttgtacacaccgcccgtcacaccatgggagtcagtaacgcccgaagccggtgacccaacccgcaagggagggagccgtcgaaggtgggaccgataactggggtgaagtcgtaacaaggtagccgtatcggaaggtgcggctggatcacctccttc

SEQ ID NO: 5 - DNA, 20 bp, synthetic construct
  misc_feature 1..20: note = source = /note="Description of Artificial Sequence: Synthetic primer"
  source 1..20: mol_type = other DNA
agagtttgatcmtggctcag

SEQ ID NO: 6 - DNA, 19 bp, synthetic construct
  misc_feature 1..19: note = source = /note="Description of Artificial Sequence: Synthetic primer"
  source 1..19: mol_type = other DNA
gtgccagcmgccgcggtaa

SEQ ID NO: 7 - DNA, 20 bp, synthetic construct
  misc_feature 1..20: note = source = /note="Description of Artificial Sequence: Synthetic primer"
  source 1..20: mol_type = other DNA
cggttaccttgttacgactt

SEQ ID NO: 8 - DNA, 1657 bp, Helicobacter sp.
  source 1..1657: mol_type = genomic DNA
agagtttgatcctggctcagagtgaacgctggcggcgtgcctaatacatgcaagtcgaacgatgaaacttctagcttgctagaagtggattagtggcgcacgggtgagtaatgcataggtaacatgccctttagtctgggatagccactggaaacggtgattaatactggatactccctacgggggaaaggggctttcaataaagaatttctctttttagtgttttgtgttgttggcacaaaattctagtatttggaatgagaaattggtgttgtgaagcaatttgtgcggagattagacttagtgtctgtcgtgtcagcaaattgcgaactcatcgatttatcatccaaagacgaattttttattgaaagccttcgctaaaggattggcctatgtcctatcagcttgttggtgaggtaatggctcaccaaggctatgacgggtatccggcctgagagggtgatcggacacactggaactgagacacggtccagactcctacgggaggcagcagtagggaatattgctcaatgggggaaaccctgaagcagcaacgccgcgtggaggatgaaggttttaggattgtaaactccttttgtaagagaagattatgacggtatcttacgaataagcaccggctaactccgtgccagcagccgcggtaatacggagggtgcaagcgttactcggaatcactgggcgtaaagagcgcgtaggcgggtggtcaagtcagatgtgaaatcctgtagcttaactacagaactgcatttgaaactgaccatctagagtatgggagaggtaggtggaattcttggtgtaggggtaaaatccgtagagatcaagaggaatactcattgcgaaggcgacctgctggaacattactgacgctgatgcgcgaaagcgtggggagcaaacaggattagataccctggtagtccacgccctaaacgatgaatgctagttgttgtgaggcttgtccttgcagtaatgcagctaacgcattaagcattccgcctggggagtacggtcgcaagattaaaactcaaaggaatagacggggacccgcacaagcggtggagcatgtggtttaattcgatgatacgcgaagaaccttacctaggcttgacattgatagaatctactagagatagtggagtgcccttttagggagcttgaaaacaggtgctgcacggctgtcgtcagctcgtgtcgtgagatgttgggttaagtcccgcaacgagcgcaaccctcgtccttagttgctagcagtttggctgagcactctaaggagactgccttcgtaaggaggaggaaggtgaggacgacgtcaagtcatcatggcccttacgcctagggctacacacgtgctacaatggggtgcacaaagagatgcaatagtgtgagctggagccaatctctaaaacatctctcagttcggattgtagtctgcaactcgactacatgaagctggaatcgctagtaatcgcaaatcagcaatgttgcggtgaatacgttcccgggtcttgtactcaccgcccgtcacaccatgggagttgtatttgccttaagtcggaatgctaaattggctaccgcccacggcagatgcagcgactggggtgaagtcgtaacaaggtaaccgtaggtgaacctgcggttg

SEQ ID NO: 9 - DNA, 1340 bp, Campylobacter sp.
  source 1..1340: mol_type = genomic DNA
agtgaacgctggcggcgtgcctaatacatgcaagtcgaacgatgaagcttctagcttgctagaagtggattagtggcgcacgggtgagtaaggtatagttaatctgccctacacaagaggacaacacctagaaatgggtgctaatactctatactcctgcttaacacaagttgagtagggaaagtttttcggtgtaggatgagactatatagtatcagctagttggtaaggtaaaggcttaccaaggctatgacgcttaagaggtctgagaggatgatctctcacactggaactgagacacggtccagactcctacgggaggcagcagtagggaatattgcgcaatgggcgaaagcctgacgcagcaacgccgcgtggaggatgacacttttaggagcgtaaactccttttcttagggaagaattctgacggtacctaaggaataagcaccggctaactccgtgccagcagccgcggtaatacggagggtgcaagcgttactcggaatcactgggcgtaaagggcgcgtaggcggattatcaagtctcttgtgaaatctaatggcttaaccattaaactgcttgggaaactgatagtctagagtgagggagaggcagatggaattggtggtgtaggggtaaaatccgtagatatcaccaagaatacccattgcgaaggcgatctgctggaactcaactgacgctaaggcgcgaaagcgtggggagcaaacaggattagataccctggtagtccacgccctaaacgatgtatgctagttgttgggctgctagtcagctcagtaatgcagctaacgcattaagcataccgcctggggagtacggtcgcaagattaaaactcaaaggaatagacggggacccgcacaagcggtggagcatgtggtttaattcgaagatacgcgaagaaccttacctaggcttgatatccaacaaagcttctagagatagaagtgtgctagcttgctagaatgttgagacaggtgctgcacggctgtcgtcagctcgtgtcgtgagatgttgggttaagtcccgcaacgagcgcaacccacgtatttagttgctaacacttcgggtgagcactctaaatagactgccttcgtaaggaggaggaaggtgtggacgacgtcaagtcatcatggcccttatgcctagggcgacacacgtgctacaatggcatatacaatgagacgcaataccgcgaggtggagcaaatctataaaatatgtcccagttcggattgttctctgcaactcgagagcatgaagccggaatcgctagtaatcgcaaatcagccatgttgcggtgaatacgttcccgggtct

SEQ ID NO: 10 - DNA, 1378 bp, Succinivibrio sp.
  source 1..1378: mol_type = genomic DNA
catgcaagtcgaacggtaacatagaggaagcttgctttctctgatgacgagtggcggacgggtgagtaaggtctgggaaactgcctgacagagggggacaacaactggaaacggttgctaataccgcatacaccctgagggggaaagtcgaaagacgctgtcagatgtgcccagatgggattagctagtaggtgaggtaaaggctcacctaggcgacgatctctagctggtctgagaggatgatcagccacattgggactgagacacggcccagactcctacgggaggcagcagtagggaatattgcacaatggggggaaccctgatgcagccatgccgcgtgtgtgaagaaggccttcgggttgtaaagcactttcagaggggaggaaaatgacgttaccctcagaagaagcaccggctaactccgtgccagcagccgcggtaatacggagggtgcaagcgttaatcggaataactgggcgtaaagggcatgcaggcggttctgcaagtagggtgtgaaagcccggggctcaacctcggaattgcactctaaactgtgggactagagtattgcagggggagacggaattccaggtgtagcggtggaatgcgtagagatctggaagaacaccaaaggcgaaggcagtctcctgggcaaatactgacgctcatatgcgaaagcgtgggtagcaaacaggattagataccctggtagtccacgccgtaaacgatgttgattagaagcttgcttgtaagagtgggtttcgcagctaacgcgataaatcaaccgcctggggagtacggccgcaaggttaaaactcaaatgaattgacgggggcccgcacaagcggtggagcatgtggtttaattcgacgcaacgcgatgaaccttacctgatcttgacatcgcgagaattacttgtaatgagtaagtgccttcgggaactcgcagacaggtgctgcatggctgtcgtcagctcgtgtcgtgagatgttgggttaagtcccgcaacgagcgcaacccttgtcctttgttgccagcgggtagagccgggaactcaaaggagactgccagtgataaactggaggaaggtagggatgacgtcaagtcatcatggcccttacggtcagggctacacacgtgctacaatggggcgtacagagggaaacgaaactgcgaggtggagtggaacccagaaagcgtccctaagttcggattggagtctgcaactcgactccatgaagtcggaatcgctagtaatcgcaaatcagaatgttgcggtgaatacgttcccgggccttgtacacaccgcccgtcacaccatgggagtggattgcaccagaagtggccagcctaactgcaaagagggcggtaccacg

SEQ ID NO: 11 - DNA, 253 bp, Anaerobiospirillum sp.
  source 1..253: mol_type = genomic DNA
tacggagggtgcaagcgttaatcggaataactgggcgtaaagggcatgtaggcggaaaggcaagcaagatgtgaaagacctgggctcaacctgggttggtcattttgaactacctttctagagtattgcagagggagatggaatttcaggtgtagcggtggaatgcgtagatatctgaaagaacaccagaggcgaaggcggtctcctgggcaaatactgacgctgaggtgcgaaagcgtggggagcaaacagg

SEQ ID NO: 12 - DNA, 1357 bp, Collinsella sp.
  modified_base 766: mod_base = OTHER; note = a, c, t, g, unknown or other
  source 1..1357: mol_type = genomic DNA
acggcacccctctccggagggaagcgagtggcgaacggctgagtaacacgtggagaacctgccccctcccccgggatagccgcccgaaaggacgggtaataccggatacccccgggcgccgcatggcgcccgggctaaagccccgacgggaggggatggctccgcggcccatcaggtagacggcggggtgacggcccaccgtgccgacaacgggtagccgggttgagagaccgaccggccagattgggactgagacacggcccagactcctacgggaggcagcagtggggaatcttgcgcaatggggggaaccctgacgcagcgacgccgcgtgcgggacggaggccttcgggtcgtaaaccgctttcagcagggaagagtcaagactgtacctgcagaagaagccccggctaactacgtgccagcagccgcggtaatacgtagggggcgagcgttatccggattcattgggcgtaaagcgcgcgtaggcggcccggcaggccgggggtcgaagcggggggctcaaccccccgaagcccccggaacctccgcggcttgggtccggtaggggagggtggaacacccggtgtagcggtggaatgcgcagatatcgggtggaacaccggtggcgaaggcggccctctgggccgagaccgacgctgaggcgcgaaagctgggggagcgaacaggattagataccctggtagtcccagccgtaaacgatggacgctgggtgtggggggacgatccccccgtgccgcagccnacgcattaagcgtcccgcctggggagtacggccgcaaggctaaaactcaaaggaattgacgggggcccgcacaagcagcggagcatgtggcttaattcgaagcaacgcgaagaaccttacggcgcatccccccgaggcccacggggggtccgccgcgtgggtcagaggagcgcatacgggaggtgcatggttgtcgtcagctcgtgtcgtgagatgttgggttaagtcccgcaacgagcgcaacccccgccgcgtgttgccatcgggtgatgccgggaacccacgcgggaccgccgccgtcaaggcggaggagggcggggacgacgtcaagtcatcatgccccttatgccctgggctgcacacgtgctacaatggccggtacagagggatgccaccccgcgagggggagcggatcccggaaagccggccccagttcggattgggggctgcaacccgcccccatgaagtcggagttgctagtaatcgcggatcagcatgccgcggtgaatgcgttcccgggccttgtacacaccgcccgtcacaccacccgagtcgtctgcacccgaagtcgccggcccaaccgcaaggggg

SEQ ID NO: 13 - DNA, 1454 bp, Clostridium sp.
  modified_base 635: mod_base = OTHER; note = a, c, t, g, unknown or other
  modified_base 704: mod_base = OTHER; note = a, c, t, g, unknown or other
  source 1..1454: mol_type = genomic DNA
tgagtttgatcatggctcaggacgaacgctggcggcgtgcctaacacatgcaagtcgagcgatgaaattttcttcggaaaatggattagcggcggacgggtgagtaacacgtgggtaacctgccctatagagagggatagccttccgaaagggagattaatacctcataatatcctagtatcgcatgatacatggattaaaggagcaatccgctataggatggacccgcggcgcattagctagttggtgaggtaacggctcaccaaggcgacgatgcgtagccgacctgagagggtgatcggccacattgggactgagacacggcccagactcctacgggaggcagcagtggggaatattgcacaatgggggaaaccctgatgcagcaacgccgcgtgagtgatgacggtcttcggattgtaaagctctgtctttagggacgataatgacggtacctaaggaggaagccacggctaactacgtgccagcagccgcggtaatacgtaggtggcaagcgttgtccggatttactgggcgtaaagggagcgtaggcggatctttaagtgggatgtgaaatactcgggctcaacctgggggctgcattccaaactggggatctagagtacaggaggggngagtggaattcctagtgtagcggtgaaatgcgtagagattaggaagaacaccagtggcgaaggcgactntctggactgtaactgacgctgaggctcgaaagcgtggggagcaaacaggattagataccctggtagtccacgccgtaaacgatgaatactaggtgtagggggtgtcaactccccctgtgccgccgctaacgcattaagtattccgcctggggagtacggtcgcaagattaaaactcaaaggaattgacgggggcccgcacaagtagcggagcatgtggtttaattcgacgcaacgcgaagaaccttacctagacttgacatcttctgcattacccttaatcggggaagttccttcggggacagaatgacaggtggtgcatggttgtcgtcagctcgtgtcgtgagatgttgggttaagtcccgcaacgagcgcaacccttaagcttagttgccatcattaagttgggcactctaagttgactgccggtgacaaaccggaggaaggtggggatgacgtcaaatcatcatgccccttatgtctagggctacacacgtgctacaatggcaagtacaaagagaagcaatactgtgaagtggagcaaaactcaaaaacttgtctcagttcggattgtaggctgaaactcgcctacatgaagctggagttgctagtaatcgcgaatcagaatgtcgcggtgaatacgttcccgggtcttgtacacaccgcccgtcacaccatgagagttggcaatacccgaagtccgtaagctaaccgtaaggaggcagcggccgaaggtagggtcagcgatgggg

SEQ ID NO: 14 - DNA, 253 bp, Clostridium sp.
  source 1..253: mol_type = genomic DNA
tacgtaggtggcgagcgttatccggatttactgggcgtaaagggagcgtaggcggatgattaagtgggatgtgaaatacccgggctcaacttgggtgctgcattccaaactggttatctagagtgcaggagaggagagtggaattcctagtgtagcggtgaaatgcgtagagattaggaagaacaccagtggcgaaggcgactctctggactgtaactgacgctgaggctcgaaagcgtggggagcaaacagg

SEQ ID NO: 15 - DNA, 1403 bp, Allisonella sp.
  source 1..1403: mol_type = genomic DNA
agagtttgatcctggctcaggacgaacgctggcggcatgcttaacacatgcaagtcgaacggactgattccttcgggatgaaagttagtggcgaacgggtgagtaatgtatgagcaacctgcctctgtcaacgggataacagttggaaacgactgctaatacggtatatgaccacggcaccgcatggtgcagcggtaaaagattttatcggacagagatgggctcatatcccattaggtagttggtgagataacagcccaccaagccgacgatcagtagccggtctgagaggatgaacggccacactggaactgagacacggtccagactcctacgggaggcagcagtggggaatcttccgcaatggacgaaagtctgacggagcaacgccgcgtgaacgatgaaggtcttcggattgtaaagttctgtgatccgggacgaaggcattgattgagaacattgattgatgttgacggtaccggaaaagcaagccacggctaactacgtgccagcagccgcggtaatacgtaggtggcaagcgttgtccggaattattgggcgtaaagcgcgcgcaggcggccgtgcaagtccatcttaaaagcgtggggcttaaccccatgaggggatggaaactgcagggctggagtgtcggaggggaaagtggaattcctagtgtagcggtgaaatgcgtagagattaggaagaacaccggtggcgaaggcgactttctagacgacaactgacgctgaggcgcgaaagcgtggggagcaaacaggattagataccctggtagtccacgccgtaaacgatggatactaggtgtaggaggtatcgaccccttctgtgccggagttaacgcaataagtatcccgcctgggaagtacgatcgcaagattaaaactcaaaggaattgacgggggcccgcacaagcggtggagtatgtggtttaattcgacgcaacgcgaagaaccttaccaagccttgacattgatcgcaatccgcagaaatgcggagttcctcttcggaggacgagaaaacaggtggtgcacggctgtcgtcagctcgtgtcgtgagatgttgggttaagtcccgcaacgagcgcaacccctatcttctgttgccagcacgtaaaggtgggaactcaggagagaccgccgcggacaacgcggaggaaggcggggatgacgtcaagtcatcatgccccttatggcttgggctacacacgtactacaatgggtgcaaacaaagagaagcgaagtcgcgagatggagcggacctcataaacgcactcccagttcagattgcaggctgcaacccgcctgcatgaagtaggaatcgctagtaatcgcgggtcagcataccgcggtgaatacgttcccgggccttgtacacaccgcccgtca

SEQ ID NO: 16 - DNA, 1375 bp, Tyzzerella sp.
  source 1..1375: mol_type = genomic DNA
ctggctcaggatgaacgctggcggcgtgcttaacacatgcaagtcgaacgaagagggttagaatgagagcttcggcaggatttctttccatcttagtggcggacgggtgagtaacgtgtgggcaacctgccctgtactgggggataatcattggaaacgatgactaataccgcatgtggttctcggaaggcatcttctgaggaagaaaggatttattcggtacaggatgggcccgcatctgattagctagttggtgagataacagcccaccaaggcgacgatcagtagccgacctgagagggtgatcggccacattgggactgagacacggcccaaactcctacgggaggcagcagtggggaatattgcacaatgggcgaaagcctgatgcagcaacgccgcgtgaaggatgaagggtttcggctcgtaaacttctatcaatagggaagaaacaaatgacggtacctaaataagaagccccggctaactacgtgccagcagccgcggtaatacgtagggggcaagcgttatccggaattactgggtgtaaagggagcgtaggcggcatggtaagccagatgtgaaagccttgggcttaacccgaggattgcatttggaactatcaagctagagtacaggagaggaaagcggaattcctagtgtagcggtgaaatgcgtagatattaggaagaacaccagtggcgaaggcggctttctggactgaaactgacgctgaggctcgaaagcgtggggagcaaacaggattagataccctggtagtccacgccgtaaacgatgagtgctaggtgtcggggaggaatcctcggtgccgtagctaacgcaataagcactccacctggggagtacgaccgcaaggttgaaactcaaaggaattgacgggggcccgcacaagcggtggagcatgtggtttaattcgaagcaacgcgaagaaccttaccaaggcttgacatcccgatgaccgtcctagagataggacttctcttcggagcatcggtgacaggtggtgcatggttgtcgtcagctcgtgtcgtgagatgttgggttaagtcccgcaacgagcgcaacccttgtcactagttgctacgaaagggcactctagtgagactgccggtgacaaaccggaggaaggtggggatgacgtcaagtcctcatggcccttatgggtagggcttcacacgtcatacaatggtcggaacagagggcagcgaagccgtgaggcggagccaatcccagaaaaccgatcgtagtccggattgcagtctgcaactcgactgcatgaagtcggaatcgctagtaatcgcggatcagcatgccgcggtgaatacgttcccgggtcttgtacacaccgcccgta

SEQ ID NO: 17 - DNA, 1410 bp, Bacteroides sp.
  source 1..1410: mol_type = genomic DNA
ggcgcacgggtgagtaacacgtatccaacctgccgataactcggggatagcctttcgaaagaaagattaatacccgatggcatgtaaagacctcctggtctttacattaaagaatttcggttatcgatggggatgcgttccattagatagtaggcggggtaacggcccacctagtccacgatggataggggttctgagaggaaggtcccccacattggaactgagacacggtccaaactcctacgggaggcagcagtgaggaatattggtcaatggacgcgagtctgaaccagccaagtagcgtgaaggaagactgccctatgggttgtaaacttcttttatacgggaataaagtattccacgtgtgggattttgtatgtaccgtatgaataaggatcggctaactccgtgccagcagccgcggtaatacggaggatccgagcgttatccggatttattgggtttaaagggagcgtaggtggaagattaagtcagcctgtgaaagtttgcggcttaaccgtaaaattgcagttgatactggttttcttgagtgcagtagaggtgggcggaattcgtggtgtagcggtgaaatgcttagatatcacgaagaactccgattgcgaaggcagctcactggactgtaactgacactgatgctcgaaagtgtgggtatcaaacaggattagataccctggtagtccacacagtaaacgatgaatactcgctgtttgcgatatacagtaagcggccaagcgaaagcgttaagtattccacctggggagtacgccggcaacggtgaaactcaaaggaattgacgggggcccgcacaagcggaggaacatgtggtttaattcgatgatacgcgaggaaccttacccgggcttaaattacacctgaatagattggaaacattttagccgcaaggcaggtgtgaaggtgctgcatggttgtcgtcagctcgtgccgtgaggtgtcggcttaagtgccataacgagcgcaacccttatcttcagttactaacagttatagctgaggactctgaagagactgccgtcgtaagatgtgaggaaggtggggatgacgtcaaatcagcacggcccttacgtccggggctacacacgtgttacaatggggggtacagaaggctgctacctggcgacaggatgccaatccttaaatcctctctcagttcggactggagtctgcaacccgactccacgaagctggattcgctagtaatcgcgcatcagccatggcgcggtgaatacgttcccgggccttgtacacaccgcccgtcaagccatgaaagccgggggtacctgaagtgcgtaaccgcaaggagcgtcctagggtaaaactggtaattggggctaagtcgtaacaaggtagccgtaccggaaggtgcggctg

SEQ ID NO: 18 - DNA, 1394 bp, Parabacteroides sp.
  source 1..1394: mol_type = genomic DNA
agagtttgatcctggctcaggatgaacgctagcgacaggcttaacacatgcaagtcgaggggcagcatgatttgtagcaatacagattgatggcgaccggcgcacgggtgagtaacgcgtatgcaacttacctatcagagggggatagcccggcgaaagtcggattaataccccataaaacaggggtcccgcatgggaatatttgttaaagattcatcgctgatagataggcatgcgttccattaggcagttggcggggtaacggcccaccaaaccgacgatggataggggttctgagaggaaggtcccccacattggtactgagacacggaccaaactcctacgggaggcagcagtgaggaatattggtcaatggccgagaggctgaaccagccaagtcgcgtgaaggaagaaggatctatggtctgtaaacttcttttataggggaataaagtggaggacgtgtccttttttgtatgtaccctatgaataagcatcggctaactccgtgccagcagccgcggtaatacggaggatgcgagcgttatccggatttattgggtttaaagggtgcgtaggtggtgatttaagtcagcggtgaaagtttgtggctcaaccataaaattgccgttgaaactgggttacttgagtgtgtttgaggtaggcggaatgcgtggtgtagcggtgaaatgcatagatatcacgcagaactccgattgcgaaggcagcttactaaaccataactgacactgaagcacgaaagcgtggggatcaaacaggattagataccctggtagtccacgcagtaaacgatgattactaggagtttgcgatacaatgtaagctctacagcgaaagcgttaagtaatccacctggggagtacgccggcaacggtgaaactcaaaggaattgacgggggcccgcacaagcggaggaacatgtggtttaattcgatgatacgcgaggaaccttacccgggtttgaacgtagtctgaccggaatggaaacactccttctagcaatagcagattacaaggtgctgcatggttgcctcaactccggcccggaaggtccggcttaattgccataacaagcgcacccttttaccaaggttcaaacaggtgaagcttgaagactctgtggaacctcccccctaacctgtgagaagaagtggggatacactcaataaaccacggcccttaatcccggggggaacactggttacaatgggttgggaaagggggcttcctggcgacaggatgctaatctccaaaccatgtctcagttcggatcggagtctgcaactcgactccgtgaagctggattcgctagtaatcgcgcatcagccatggcgcggtgaatacgttcccgggccttgtacacaccgcccgtc

SEQ ID NO: 19 - DNA, 1451 bp, Bacteroides sp.
  source 1..1451: mol_type = genomic DNA
gatgaacgctagctacaggcttaacacatgcaagtcgaggggcagcatggtcttagcttgctaaggctgatggcgaccggcgcacgggtgagtaacacgtatccaacctgccgtctactcttggccagccttctgaaaggaagattaatccaggatgggatcatgagttcacatgtccgcatgattaaaggtattttccggtagacgatggggatgcgttccattagatagtaggcggggtaacggcccacctagtcaacgatggataggggttctgagaggaaggtcccccacattggaactgagacacggtccaaactcctacgggaggcagcagtgaggaatattggtcaatgggcgcgagcctgaaccagccaagtagcgtgaaggatgactgccctatgggttgtaaacttcttttgtccgggaataaaaccgcctacgtgtaggcgcttgtatgtaccggtacgaataagcatcggctaactccgtgccagcagccgcggtaatacggaggatgcgagcgttatccggatttattgggtttaaagggagcgcagacgggtttttaagtcagctgtgaaagtttggggctcaaccttaaaattgcagttgatactggagaccttgagtgcagttgaggcaggcggaattcgtggtgtagcggtgaaatgcttagatatcacgaagaactccgattgcgaaggtagcttgctaaagtgtaactgacgttcatgctcgaaagtgtgggtatcaaacaggattagataccctggtagtccacacggtaaacgatggatactcgctgttggcgatatacggtcagcggcttagcgaaagcgttaagtatcccacctggggagtacgccggcaacggtgaaactcaaaggaattgacgggggcccgcacaagcggaggaacatgtggtttaattcgatgatacgcgaggaaccttacccgggcttaaattgcactggactattctggaaacaggatattcttcggaccagtgtgaaggtgctgcatggttgtcgtcagctcgtgccgtgaggtgtcggcttaagtgccataacgagcgcaacccttgctgccagttactaacaggtaatgctgaggactctggcgggactgccatcgtaagatgcgaggaaggtggggatgacgtcaaatcagcacggcccttacgtccggagctacacacgtgttacaatggtaggtacagagggtagctacccagcgatgggatgcgaatctcgaaagcctatctcagttcggattggaggctgaaacccgcctccatgaagttggattcgctagtaatcgcgcatcagccatggcgcggtgaatacgttcccgggccttgtacacaccgcccgtcaagccatgggagccgggggtacctgaagtacgtaaccgcaaggatcgtcctagggtaaaactggtgactgggg

SEQ ID NO: 20 - DNA, 1450 bp, Bacteroides sp.
  source 1..1450: mol_type = genomic DNA
gatgaacgctagctacaggcttaacacatgcaagtcgaggggcagcatgaagtttgcttgcaaactttgatggcgaccggcgcacgggtgagtaacgcgtatccaacctcccgcatactcggggatagccttctgaaaggaagattaatacccgatggtatcttaagcgcacatgcaattaagattaaagaatttcggtatgcgatggggatgcgttccattaggtagtaggcggggtaacggcccacctagccatcgatggataggggttctgagaggaaggtcccccacattggaactgagacacggtccaaactcctacgggaggcagcagtgaggaatattggtcaatgggcgcgagcctgaaccagccaagtagcgtgaaggatgactgccctatgggttgtaaacttcttttgtccgggaataaaaccgcctacgtgtaggcgcttgtatgtaccggtacgaataagcatcggctaactccgtgccagcagccgcggtaatacggaggatgcgagcgttatccggatttattgggtttaaagggagcgcagacgggtttttaagtcagctgtgaaagtttggggctcaaccttaaaattgcagttgatactggagaccttgagtgcagttgaggcaggcggaattcgtggtgtagcggtgaaatgcttagatatcacgaagaactccgattgcgaaggcagcttgctaaagtgtaactgacgttcatgctcgaaagtgtgggtatcaaacaggattagataccctggtagtccacacggtaaacgatggatactcgctgttggcgatatacggtcagcggcttagcgaaagcgttaagtatcccacctggggagtacgccggcaacggtgaaactcaaaggaattgacgggggcccgcacaagcggaggaacatgtggtttaattcgatgatacgcgaggaaccttacccgggcttaaattgcactggactttcccggaaacgggattttcttcggaccagtgtgaaggtgctgcatggttgtcgtcagctcgtgccgtgaggtgtcggcttaagtgccataacgagcgcaacccttgctgccagttactaacaggtaatgctgaggactctggcgggactgccatcgtaagatgcgaggaaggtggggatgacgtcaaatcagcacggcccttacgtccggggctacacacgtgttacaatggggggtacagaaggccgctacccggcaacgggatgccaatctccaaaacccctctcagttcggactggagtctgcaacccgactccacgaagctggattcgctagtaatcgcgcatcagccacggcgcggtgaatacgttcccgggccttgtacacaccgcccgtcaagccatgaaagccgggggtacctgaagtgcgtaaccgcaaggagcgccctagggtaaaactggtaattggggct

SEQ ID NO: 21 - DNA, 1511 bp, Bacteroides sp.
  source 1..1511: mol_type = genomic DNA
agagtttgatcctggctcaggatgaacgctagctacaggcttaacacatgcaagtcgaggggcagcgggattgaagcttgcttcaattgccggcgaccggcgcacgggtgagtaacgcgtatccaaccttccgcttactcggggatagcctttcgaaagaaagattaatacccgatggtatcttaagcacgcatgagattaagattaaagatttatcggtaagcgatggggatgcgttccattaggcagttggcggggtaacggcccaccaaacctacgatggataggggttctgagaggaaggtcccccacattggaactgagacacggtccaaactcctacgggaggcagcagtgaggaatattggtcaatgggcgagagcctgaaccagccaagtagcgtgaaggatgacggccctacgggttgtaaacttcttttgtgcgggaataaaggaacctacgtgtaggtttttgcatgtaccgtaacgaataagcatcggctaactccgtgccagcagccgcggtaatacggaggatgcgagcgttatccggatttattgggtttaaagggagcgtagacgggtttttaagtcagctgtgaaagtttggggctcaaccttaaaattgcagttgaaactggagaccttgagtacggttgaggcaggcggaattcgtggtgtagcggtgaaatgcttagatatcacgaagaaccccgattgcgaaggcagcctgctaagccgccactgacgttgaggctcgaaagtgcgggtatcaaacaggattagataccctggtagtccgcacggtaaacgatggatactcgctgttggcgatagacagtcagcggccaagcgaaagcgttaagtatcccacctggggagtacgccggcaacggtgaaactcaaaggaattgacgggggcccgcacaagcggaggaacatgtggtttaattcgatgatacgcgaggaaccttacccgggcttgaactgcagtggaattatccggaaacggataagcgagcaatcgccgctgtggaggtgctgcatggttgtcgtcagctcgtgccgtgaggtgtcggcttaagtgccataacgagcgcaacccttgctgccagttactaacaggtcatgctgaggactctggcaggactgccatcgtaagatgcgaggaaggtggggatgacgtcaaatcagcacggcccttacgtccggggctacacacgtgttacaatggggagtacagagggcagctaccgggcgaccggatgcgaatcccgaaagctcctctcagttcggactggagtctgcaacccgactccacgaagctggattcgctagtaatcgcgcatcagccacggcgcggtgaatacgttcccgggccttgtacacaccgcccgtcaagccatgaaagccgggggtacctgaagtacgtaaccgcgaggatcgtcctagggtaaaaccggtaattggggctaagtcgtaacaaggtagccgtaccggaaggtgcggctg

SEQ ID NO: 22 - DNA, 1491 bp, Blautia sp.
  source 1..1491: mol_type = genomic DNA
agagtttgatcctggctcaggatgaacgctggcggcgtgcttaacacatgcaagtcgaacgagaaacattttaatgaagcttcggcagatttagtttgtttctagtggcggacgggtgagtaacgcgtgggtaacctgcctcacactgggggataacagtcagaaatgactgctaataccgcataagcgcacggaaccgcatggttttgtgtgaaaaactccggtggtgtgagatggacccgcgttggattagccagttggcagggtaacggcctaccaaagcgacgatccatagccggcctgagagggtgaacggccacattgggactgagacacggcccagactcctacgggaggcagcagtggggaatattgcacaatgggggaaaccctgatgcagcgacgccgcgtgaaggaagaagtatctcggtatgtaaacttctatcagcagggaagataatgacggtacctgactaagaagccccggctaactacgtgccagcagccgcggtaatacgtagggggcaagcgttatccggatttactgggtgtaaagggagcgtagacggagcagcaagtctgatgtgaaaggcaggggctcaacccctggactgcattggaaactgttgatcttgagtaccggaggggtaagcggaattcctagtgtagcggtgaaatgcgtagatattaggaggaacaccagtggcgaaggcggcttactggacggtaactgacgttgaggctcgaaagcgtggggagcaaacaggattagataccctggtagtccacgccgtaaacgatgaatactaggtgtcgggtggcagagccattcggtgccgcagcaaacgcagtaagtattccacctggggagtacgttcgcaagaatgaaactcaaaggaattgacggggacccgcacaagcggtggagcatgtggtttaattcgaagcaacgcgaagaaccttaccaagtcttgacatccctctgaccggtccttaaccggacctttccttcgggacagaggagacaggtggtgcatggttgtcgtcagctcgtgtcgtgagatgttgggttaagtcccgcaacgagcgcaacccctatccccagtagccagcatttaaggtgggcactctgaggagactgccagggataacctggaggaaggcggggatgacgtcaaatcatcatgccccttatgatttgggctacacacgtgctacaatggcgtaaacaaagggaagcagagcggtgacgccgagcaaatcccaaaaataacgtcccagttcggactgcagtctgcaactcgactgcacgaagctggaatcgctagtaatcgcggatcagaatgccgcggtgaatacgttcccgggtcttgtacacaccgcccgtcacaccatgggagtcagtaacgcccgaagtcagtgacctaaccgaaagggaggagctgccgaaggcgggacggatgactggggtgaagtcgtaacaaggtaacc

SEQ ID NO: 23 - DNA, 1336 bp, Fusobacterium sp.
  source 1..1336: mol_type = genomic DNA
gatgaacgctgacagaatgcttaacacatgcaagtctacttgaattcacttcggtgatagtaaggtggcggacgggtgagtaacacgtaaagaacttgccttacagtctgggacaactattggaaacgatagctaataccggatattatgcgagagtcgcatgactcttgtatgaaagctatatgcgctgtaagagagctttgcgtcccattagctagttggtgaggtaacggctcaccaaggccacgatgggtagccggcctgagagggtgaacggccacaaggggactgagacacggcccttactcctacgggaggcagcagtggggaatattggacaatggaccaaaagtctgatccagcaattctgtgtgcacgatgacggtcttaggattgtaaagtgctttcaattgggaagaaaaaaatgacggtaccaatagaagaagcgacggctaaatacgtgccagcagccgcggtaatacgtatgtcgcaagcgttatccggatttattgggcgtaaagcgcgtctaggtggtttggtaagtctgatgtgaaaatgcggggctcaactccgtattgcgttggaaactgcctaactagagtatcggagaggtgggcggaactacaagtgtagaggtgaaattcgtagatatttgtaggaatgccgatagagaagtcagctcactggacgaatactgacactgaagcgcgaaagcatggggagcaaacaggattagataccctggtagtccatgctgtaaacgatgattactaagcgtcgggggtcgaacctcggcactcaagctaacgcgataagtaatccgcctggggagtacgtacgcaagtatgaaactcaaaggaattgacggggacccgcacaagtggtggagcatgtggtttaattcgacgcaacgcgaggaaccttaccagcgtttgacatcctaggaatgagaaagagatttcttagtgctccttcgggagaacctagagacaggtggtgcatggctgtcgtcagctcgtgtcgtgagatgttgggttaagtcccgcaacgagcgcaacccctattgtatgttgccatcattaagttgggcactcatgcgatactgcctgcgatgagcaggaggaaggtggggatgacgtcaagtcatcatgccccttatacgctgggctacacacgtgctacaatgggcagtacagagagaagcaaatctgcgaggaggagcaaatctcacaaagctgttcgtagttcggattgtactctgcaactcgagtacatgaagttggaatcactagtaatcgcaaatcagctatgttgcggtgaatacgttctcgggtct

SEQ ID NO: 24 - DNA, 1359 bp, unidentified
  misc_feature 1..1359: note = "source /noteDescription of Unknown: Lachnospiraceae sequence"
  source 1..1359: mol_type = genomic DNA
gatgaacgctggcggcgtgcttaacacatgcaagtcgaacgggaaacattttaatgaagcttcggcagatttagcttgtttctagtggcggacgggtgagtaacgcgtgggtaacctgcctcacactgggggataacagtcagaaatgactgctaataccgcataagcgcacggaaccgcatggttttgtgtgaaaaactccggtggtgtgagatggacccgcgttggattagccagttggcagggtaacggcctaccaaagcgacgatccatagccggcctgagagggtgaacggccacattgggactgagacacggcccagactcctacgggaggcagcagtggggaatattgcacaatgggggaaaccctgatgcagcgacgccgcgtgaaggaagaagtatctcggtatgtaaacttctatcagcagggaagaaaatgacggtacctgactaagaagccccggctaactacgtgccagcagccgcggtaatacgtagggggcaagcgttatccggatttactgggtgtaaagggagcgtagacggaatggcaagtctgatgtgaaaggcaggggctcaacccctggactgcattggaaactgtcagtcttgagtaccggaggggtaagcggaattcctagtgtagcggtgaaatgcgtagatattaggaggaacaccagtggcgaaggcggcttactggacggtaactgacgttgaggctcgaaagcgtggggagcaaacaggattagataccctggtagtccacgccgtaaacgatgaatacgaggtgtcgggtgggcaaagccattcggtgccgcagcaaacgcaaaaagtaatcccacctgggggagtacgttcccaagaatgaaactcaaaggaaatagcggggacccgcacaagcggtggagcatgtggtgtatttgaagcaacgcgaagaaccttaccaagtcttgacatccctctgaccggtccttaaccggacctctccttcgggacaggggagacaggtggtgcatggttgtcgtcagctcgtgtcgtgagatgttgggttaagtcccgcaacgagcgcaacccctatccttagtagccagcatctgaggtgggcactctgaggagactgccagggataacctggaggaaggcggggaggacgtcaaatcatcatgccccctatgatttgggctacacacgtgctacaatggcgtaaacaaagggaagcagagcggtgacgccgagcaaatcccaaaaataacgtcccagttcggactgcagtctgcaactcgactgcacgaagctggaatcgctagtaatcgcggatcagaatgccgcggtgaataaaagcccgggtcttgcact

SEQ ID NO: 25 - DNA, 1387 bp, Blautia sp.
  source 1..1387: mol_type = genomic DNA
agagtttgatcatggctcaggatgaacgctggcggcgtgcttaacacatgcaagtcgaacgggaattactttattgaagctttggtcgatttaatttaattatagtggcggacgggtgagtaacgcgtgggtaacctgccttatacagggggataacagtcagaaatggctgctaataccgcataagcgcacagagctgcatggctcagtgtgaaaaactccggtggtataagatggacccgcgttggattagttggttggtggggtaacggcccaccaaggcgacgatccatagccggcctgagagggtgaacggccacattgggactgagacacggcccagactcatacgggaggcagcagtggggaatattgcacaatgggggaaaccctgatgcagcgacgccgcgtgaaggaagaagtatctcggtatgtaaacttctatcagcagggaagatagtgacggtacctgactaagaagccccggctaactacgtgccagcagccgcggtaatacgtagggggcaagcgttatccggatttactgggtgtaaagggagcgtagacggtgtggcaagtctgatgtgaaaggcatgggctcaacctgtggactgcattggaaactgtcatacttgagtgccggaggggtaagcggaattcctagtgtagcggtgaaatgcgtagatattaggaggaacaccagtggcgaaggcggcttactggacggtaactgacgttgaggctcgaaagcgtggggagcaaacaggattagataccctggtagtccacgccgtaaacgatgaatactaggtgtcgggtggcaaagccattcggtgccgtcgcaaacgcagtaagtattccacctggggagtacgttcgcaagaatgaaactcaaaggaattgacggggacccgcacaagcggtggagcatgtggtttaattcgaagcaacgcgaagaaccttaccaagtcttgacatccgcctgaccgatccttaaccggatctttccttcgggacaggcgagacaggtggtgcatggttgtcgtcagctcgtgtcgtgagatgttgggttaagtcccgcaacgagcgcaacccctatcctcagtagccagcattaagttgggcactcatgcgatactgcctgcgatgagcaggaggaaggtggggatgacgtcaagtcatcatgccccttatacgctgggctacacacgtgctacaatgggtagtacagagagtcgcaaacctgcgagggggagctaatctcagaaaactattctcagttcggattgtactctgcaactcgagtacatgaagttggaatcgctagtaatcgcaaatcagctatgttgcggtgaatacgttctcgggtcttgcactcaccgcccgt

SEQ ID NO: 26 - DNA, 1332 bp, Blautia sp.
  source 1..1332: mol_type = genomic DNA
gctcaggatgaacgctggcggcgtgcttaacacatgcaagtcgagcgaagcacttgccattgactcttcggaagatttggcatttgactgagcggcggacgggtgagtaacgcgtgggtaacctgcctcatacgggggaataacagttagaaatggctgctaatgccgcataaccgcacaggaccgcatggactggtgtgaaaaactgaggtggtatgagatgggcccgcgtctgattaggttagttggcggggtaacggcccaccaagccgacgatcagtagccgacctgagagggaccggccacattgggactgagacatggcccagactcctacgggaggcagcagtggggaatattgcacaatggaggaaactctgatgcagcgacgccgcatgaaggaagaagtatctcggtatgtaaacttctatcagcagggaagaaaatgacggtacctgactaagaagccccggctaactacgtgccagcagccgcggtaatacgtagggggcaagcgttatccggatttactgggtgtaaagggagcgtagacggacgggcaagtctgatgtgaaagcccggggcttaaccccgggactgcattggaaactgtccatcttgagtgccggagaggtaagcggaattcctagtgtagcggtgaaatgcgtagatattaggaggaacaccagtggcgaaggcggcttactggacggtaactgacgttgaggctcgaaagcgtggggagcaaacaggattagataccctggtagtccacgccgtaaacgatcaataatgggtgtcgggttgcaaagcaatccggtgccgcagcaaacgcagtaagtattccccctcgggagtacgttcgcaagaatgaaactcaaaggaagggacggggatccgcacaagcggcggagcatgtggtttaattagaagcaacgcgaagaaccttaccaagtcttgacatctgcctgaccgttccttaaccggaactatctttcgggacaggcaagacaggtggtgcatggttgtcgtcagctcgtgtcgtgagatgttgggttaagtcccgcaacgagcgcaacccctgtccttagtagccagcagtccggctgggcactctagggagactgccgggggtaacccggaggaaggcggggaggaggtcaaatcatcatgccccccctgatttgggctacacacgtggtacaatggcgtaaacaaagggaagcggagtggtgacgctgagcaaatctcaaaaataacgtcccacttcggactgcagtctgcaactcgactgcacgaagctggaatcgctagtaatcgcgaatcagaatg

SEQ ID NO: 27 - DNA, 253 bp, Blautia sp.
  source 1..253: mol_type = genomic DNA
tacgtagggggcaagcgttatccggatttactgggtgtaaagggagcgtagacggcatggcaagtctgatgtgaaaggcaggggctcaactcctggactgcattggaaactgccaggcttgagtgccggaggggtaagcggaattcctagtgtagcggtgaaatgcgtagatattaggaggaacaccagtggcgaaggcggcttactggacggtaactgacgttgaggctcgaaagcgtggggagcaaacagg

SEQ ID NO: 28 - DNA, 1324 bp, Intestinibacter sp.
  source 1..1324: mol_type = genomic DNA
cgtaagtaacctgccctgtacacacggataacataccgaaaggtatgctaatacgggataatatattttgatcgcatggtcgagatatcaaagctccggcggtacaccagggacccccgacagaggagctagttggtagtaatgtcaccaaggcgacgatcagaagccgaactgagagggggatccgcacatgactgagacacggtcaaactcctacgggaggcagcagtggggaatatgccaatgggcgaaagctgatgcagcacgcgcgtgagcgatgaggctcgggtcgtaaagctcgtctcaaggaagataatgacggtacttgaggaggaagccccggctaactacgtgccagcagccgcggtaatacgtagggggctagcgttatccggaattactgggcgtaaagggtgcgtaggcggtctttcaagtcaggagtgaaaggctacggctcaaccgtagtaagctcttgaaactgtaagacttgagtgcaggagaggagagtggaattcctagtgtagcggtgaaatgcgtagatattaggaggaacaccagttgcgaaggcggctctctggactgtaactgacgctgaggcacgaaagcgtggggagcaaacaggattagataccctggtagtccacgccgtaaacgatgagtactagctgtcggaggttacccccttcggtggcgcagctaacgcattaagtactccgcctgggaagtacgctcgcaagagtgaaactcaaaggaattgacggggacccgcacaagtagcggagcatgtggtttaattcgaagcaacgcgaagaaccttacctaagcttgacatcccactgacccttccctaatcggaagcttcccttcgggacagtggtgacaggtggtgcatggttgtcgtcagctcgtgtcgtgagatgttgggttaagtcccgcaacgagcgcaacccttgcctttagttgccagcattaagttgggcactctagagggactgccagggataacccggaggagtggggatgacgtcaaatcatcatgcccttatgctaggctacacacgtgctacaatgggtggtcagaggccagccagtcgtgaggccgagctatcccataagccattctcgtccggattgtaggctgaactcgcctacatgagctggaattacaagtatgcgatcgatgctgcgtgatgcgtccgggtcttgtacacaccgcccgtcacaccatgggagttgggggcgcccgaagccggattgctaaccttttggaagcgtccgtcgaaggtgaaaccaataactggggtgaagtcgtaacaaggtaacc

SEQ ID NO: 29 - DNA, 1342 bp, Corynebacterium sp.
  source 1..1342: mol_type = genomic DNA
gacgaacgctggcggcgtgcttaacacatgcaagtcgaacggaaaggccccagctcgctggggtactcgagtggcgaacgggtgagtaacacgtgggtgatctgccttgcactctgggataagcttgggaaactgggtctaataccggatatgaactgcctttagtgtggtggttggaaagttttttcggtgcaagatgagctcgcggcctatcagcttgttggtggggtaatggcctaccaaggcgtcgacgggtagccggcctgagagggtgtacggccacattgggactgagatacggcccagactcctacgggaggcagcagtggggaatattgcacaatgggcggaagcctgatgcagcgacgccgcgtgggggatgacggccttcgggttgtaaactcctttcgacagggacgaagctttttgtgacggtacctgtataagaagcaccggctaactacgtgccagcagccgcggtaatacgtagggtgcgagcgttgtccggaattactgggcgtaaagagctcgtaggtggtttgtcgcgtcgtctgtgaaattccggggcttaactccgggcgtgcaggcgatacgggcataacttgagtactgtaggggagactggaattcctggtgtagcggtgaaatgcgcagatatcaggaggaacaccggtggcgaaggcgggtctctgggcagtaactgacgctgaggagcgaaagcatggggagcgaacaggattagataccctggtagtccatgccgtaaacggtgggcgctaggtgtgggtttccttccacgggatccgtgccgtagctaacgcattaagcgccccgcctggggagtacggccgcaaggctaaaactcaaaggaattgacgggggcccgcacaagcggcggagcatgtggattaattcgatgcaacgcgaagaaccttacctgggcttgacatacactggatcgggctagagatagtctttccctttgtggctggtgtacaggtggtgcatggttgtcgtcagctcgtgtcgtgagatgttgggttaagtcccgcaacgagcgcaacccttgtcttatgttgccagcatttggttggggactcatgagagactgccggggtcaactcggaggaaggtggggatgacgtcaaatcatcatgccccttatgtccagggcttcacacatgctacaatggtcggtacaacgcgcagcgacactgtgaggtggagcgaatcgctgaaagccggccttagttcggattggggtctgcaactcgaccccatgaagtcggagtcgctagtaatcgcagatcagcaatgctgcggtgaatacgttcccgggcct

SEQ ID NO: 30 - DNA, 253 bp, Clostridium sp.; identical to SEQ ID NO: 14
  source 1..253: mol_type = genomic DNA

SEQ ID NO: 31 - DNA, 1399 bp, Enterococcus sp.
  source 1..1399: mol_type = genomic DNA
cttgtgtcaccaaccatagggagggggaaaacatggaaacggggttcataccgcataacttttttagcccaatgcataagaagaaaggcctttcgggtttcggtaaaggaggcccccgcggctcttatagtgtgtgtggaagtaaccgcttccacaaggcccaggtttcatacccgactggagagtgtgttcgccacactggggaaaggacccccggcccagtctctctaggggaggcagcagtaggaattttcggcaaaggaaaaaatttctgaccgaacaacgccggttgaatgaagaagtttttcggatcgaaaaactctgttgttagagaagaacaaggacgttagtaactgaacgtcccctgacggtatctaaccagaaagccacggctaattacgtgccagcagccgcggtaatacgtaggtggcaagcgttgtccggatttattgggcgtaaagcgagcgcaggcggtttcttaagtctgatgtgaaagcccccggctcaaccggggagggtcattggaaactgggagacttgagtgcagaagaggagagtggaattccatgtgtagcggtgaaatgcgtagatatatggaggaacaccagtggcgaaggcggctctctggtctgtaactgacgctgaggctcgaaagcgtggggagcaaacaggattagataccctggtagtccacgccgtaaacgatgagtgctaagtgttggagggtttccgcccttcagtgctgcagcaaacgcattaagcactccgcctggggagtacgaccgcaaggttgaaactcaaaggaattgacgggggcccgcacaagcggtggagcatgtggtttaattcgaagcaacgcgaagaaccttaccaggtcttgacatcctttgaccactctagagatagagctttcccttcggggacaaagtgacaggtggtgcatggttgtcgtcagctcgtgtcgtgagatgttgggttaagtcccgcaacgagcgcaacccttattgttagttgccatcatttagttgggcactctagcgagactgccggtgacaaaccggaggaaggtggggatgacgtcaaatcatcatgccccttatgacctgggctacacacgtgctacaatgggaagtacaacgagtcgctagaccgcgaggtcatgcaaatctcttaaagcttctctcagttcggattgcaggctgcaactcgcctgcatgaagccggaatcgctagtaatcgcggatcagcacgccgcggtgaatacgttcccgggccttgtacacaccgcccgtcacaccacgagagtttgtaacacccgaagtcggtgaggtaacctttttggagccagccgcctaaggtgggatagatgattggggtgaagtcgtaaccaacgtatgcc

SEQ ID NO: 32 - DNA, 1393 bp, Streptococcus sp.
  modified_base 1381: mod_base = OTHER; note = a, c, t, g, unknown or other
  source 1..1393: mol_type = genomic DNA
agactttagcttgctaaagttggaagagttgcgaacgggtgagtaacgcgtaggtaacctgcctactagcgggggataactattggaaacgatagctaataccgcataacagcatttaacccatgttagatgcttgaaaggagcaattgcttcactagtagatggacctgcgttgtattagctagttggtgaggtaacggctcaccaaggcgacgatacatagccgacctgagagggtgatcggccacactgggactgagacacggcccagactcctacgggaggcagcagtagggaatcttcggcaatgggggcaaccctgaccgagcaacgccgcgtgagtgaagaaggttttcggatcgtaaagctctgttgtaagagaagaacgtgtgtgagagtggaaagttcacacagtgacggtaacttaccagaaagggacggctaactacgtgccagcagccgcggtaatacgtaggtcccgagcgttgtccggatttattgggcgtaaagcgagcgcaggcggtttaataagtctgaagttaaaggcagtggcttaaccattgttcgctttggaaactgttagacttgagtgcagaaggggagagtggaattccatgtgtagcggtgaaatgcgtagatatatggaggaacaccggtggcgaaagcggctctctggtctgtaactgacgctgaggctcgaaagcgtggggagcaaacaggattagataccctggtagtccacgccgtaaacgatgagtgctaggtgttaggccctttccggggcttagtgccgcagctaacgcattaagcactccgcctggggagtacgaccgcaaggttgaaactcaaaggaattgacgggggcccgcacaagcggtggagcatgtggtttaattcgaagcaacgcgaagaaccttaccaggtcttgacatcccgatgctattcctagagataggaagtttcttcggaactgtgagacttgagggcagaagggtagagtgcacttgtatggggagctgtggaatgcgttcccgcaacgagcgcaacccctattgttagttgccatcattaagttgggcactctagcgagactgccggtaataaaccggaggaaggtggggatgacgtcaaatcatcatgccccttatgacctgggctacacacgtgctacaatggttggtacaacgagtcgcgagtcggtgacggcaagcaaatctcttaaagccaatctcagttcggattgtaggctgcaactcgcctacatgaagtcggaatcgctagtaatcgcggatcagcacgccgcggtgaatacgttcccgggccttgtacacaccgcccgtcacaccacgagagtttgtaacacccgaagtcggtgaggtanccttttaggagc

SEQ ID NO: 33 - DNA, 1418 bp, Megasphaera sp.
  source 1..1418: mol_type = genomic DNA
agagtttgatcatggctcaggacgaacgctggcggcgtgcttaacacatgcaagtcgaacgagaagagatgagaagcttgcttcttatctcttcgagtggcaaacgggtgagtaacgcgtaagcaacctgcccttcagatggggacaacagctggaaacggctgctaataccgaatacgttctttttgtcgcatggcagagggaagaaagggaggctcttcggagctttcgctgaaggaggggcttgcgtctgattagctagttggaggggtaacggcccaccaaggcgacgatcagtagccggtctgagaggatgaacggccacattgggactgagacacggcccagactcctacgggaggcagcagtggggaatcttccgcaatggacgaaagtctgacggagcaacgccgcgtgaacgatgacggccttcgggttgtaaagttctgttatacgggacgaatggcgtagcggtcaatacccgttacgagtgacggtaccgtaagagaaagccacggctaactacgtgccagcagccgcggtaatacgtaggtggcaagcgttgtccggaattattgggcgtaaagggcgcgcaggcggcgtcgtaagtcggtcttaaaagtgcggggcttaaccccgtgaggggaccgaaactgcgatgctagagtatcggagaggaaagcggaattcctagtgtagcggtgaaatgcgtagatattaggaggaacaccagtggcgaaagcggctttctggacgacaactgacgctgaggcgcgaaagccaggggagcaaacgggattagataccccggtagtcctggccgtaaacgatggatactaggtgtaggaggtatcgaccccttctgtgccggagttaacgcaataagtatcccgcctggggagtacggccgcaaggctgaaactcaaaggaattgacgggggcccgcacaagcggtggaacatgtggtttaattcgatgatacgcgaggaaccttacccgggcttaaattgcagtggaatgatgtggaaacatgtcagtgagcaatcaccgctgtgaaggtgctgcatggttgtcgtcagctcgtgccgtgaggtgtcggcttaagtgccataacgagcgcaacccttatcttcagttactaacaggtcatgctgaggactctggagagactgccgtcgtaagatgtgaggaaggtggggatgacgtcaaatcagcacggcccttacgtccggggctacacacgtgttacaatggggggtacagagggccgctaccacgcgagtggatgccaatcccaaaaacctctctcagttcggactggagtctgcaacccgactccacgaagctggattcgctagtaatcgcgcatcagccacggcgcggtgaatacgttcccgggccttgcactcaccgcccgt

SEQ ID NO: 34 - DNA, 1394 bp, Parabacteroides sp.; identical to SEQ ID NO: 18
  source 1..1394: mol_type = genomic DNA

SEQ ID NO: 35 - DNA, 1472 bp, unidentified
  misc_feature 1..1472: note = source = /note="Description of Unknown: Escherichia-Shigella sequence"
  source 1..1472: mol_type = genomic DNA
cgccctgattgacggctatacacatgcaagtcgaacggtaacaggaaacagcttgcttctttgctgacgagtggcggacgggtgagtaatgtctgggaaactgcctgatggagggggataactactggaaacggtagctaataccgcataacgtcgcaagaccaaagagggggaccttcgggcctcttgccatcggatgtgcccagatgggattagctagtaggtggggtaacggctccatccctaggcgagccgaatccttagcctggtctgagaggaatgaccagccacactgggactgagaacacggtccagactcctacgggaggcagcagtggggaatattgcacaatgggcgcaagcctgatgcagccatgccgcgtgtatgaagaaggccttcgggttgtaaagtactttcagcggggaggaagggagtaaagttaataccctttgctcattgacgttacccgcagaagaagcaccggctaactccgtgccagcagccgcggtaatacggagggtgcaagcgttaatcggaattactgggcgtaaagcgcacgcaggcggtttgttaagtcagatgtgaaatccccgggctcaacctgggaactgcatctgatactggcaagcttgagtctcgtagaggggggtagaattccaggtgtagcggtgaaatgcgtagagatctggaggaataccggtggcgaaggcggccccctggacgaagactgacgctcaggtgcgaaagcgtggggagcaaacaggattagataccctggtagtccacgccgtaaacgatgtcgacttggaggttgtgcccttgaggcgtggcttccggagctaacgcgttaagtcgaccgcctggggagtacggccgcaaggttaaaactcaaatgaattgacgggggcccgcacaagcggtggagcatgtggtttaattcgatgcaacgcgaagaaccttacctggtcttgacatccacgggaagttttcagagatgagaatgtgccttcgggaaccgtgagacaggtgctgcatggctgtcgtcagctcgtgttgtgaaatgttgggttaagtcccgcaacgagcgcaacccttatcctttgttgccagcggtccggccgggaactcaaaggagactgccagtgataaactggaggaaggtggggatgacgtccaggtcatcatggcccttacgaaccagggctacacacgtgcctacaatggacgcatccaaagagagagcgaaccctgcccgcgagagcaagcggacctcataaagtgcgtcgtagtccggattggagtctgcaactcgactccatgaagtcggaatcgctagtaatcgtggatcagaatgccacggtgaatacgttcccgggccttgtacacaccgcccgtcacaccatgggagtgggttgcaaaagaagtaggtagcttaaccttcgggagggcgcttaccactttggatgcgagg

SEQ ID NO: 36 - DNA, 1440 bp, Tyzzerella sp.
  source 1..1440: mol_type = genomic DNA
taagatgaacgctggcggcgtgcttaacacatgcaagtcctatgaagcgcttaaacggatttcttcggattgaagtttttgtgactgagtggcggacgggtgagtaacgcgtgggtaacttgcctcatacagggggataacagttagaaatgactgctaataccgcataagcgcacagtgctgcatggcacagtgtgaaaaactccggtggtatgagatggacccgcgtctgattagctagttggtggggtaacggcctaccaaggcgacgatcagtagccggcctgagagggtgaacggccacattgggactgagacacggcccaaactcctacgggaggcagcagtggggaatattgcacaatgggggaaaccctgatgcagcgacgccgcgtgagcgaagaagtatttcggtatgtaaagctctatcagcagggaagaaaatgacggtacctgactaagaagcaccggctaaatacgtgccagcagccgcggtaatacgtatggtgcaagcgttatccggatttactgggtgtaaagggagcgtagacggttgtgtaagtctgatgtgaaagcccggggctcaaccccgggactgcattggaaactatgtaactagagtgtcggagaggtaagcggaattcctagtgtagcggtgaaatgcgtagatattaggaggaacaccagtggcgaaggcggcttactggacgatcactgacgttgaggctcgaaagcgtggggagcaaacaggattagataccctggtagtccacgccgtaaacgatgactactaggtgtcggggcccataagggcttcggtgccgcagcaaacgcaataagtattccacctggggagtacgttcgcaagaatgaaactcaaaggaattgacggggacccgcacaagcggtggagcatgtggtttaattcgaagcaacgcgaagaaccttacctggtcttgacatcccactgaccggacagtaatgtgtcctttcctccgggacagtggagacaggtggtgcatggttgtcgtcagctcgtgtcgtgagatgttgggttaagtcccgcaacgagcgcaacccctatccttagtagccagcagtaagatgggcactctagggagactgccagggataacctggaggaaggtggggatgacgtcaaatcatcatgccccttatgacttgggctacacacgtgctacaatggcgtaaacaaagtgaagcgaagtcgtgaggccaagcaaatcacaaaaataacgtctcagttcggattgtagtctgcaactcgactacaagaagctggaatcgctagtaatcgcagatcagaatgctgcggtgaatacgttcccgggtcttgtacacaccgcccgtcacaccatgggagtcgaaaatgcccgaagtcggtgacctaacgaaagaaggagccgccgaaggcaggtt

SEQ ID NO: 37 - DNA, 1366 bp, Fusobacterium sp.
  source 1..1366: mol_type = genomic DNA
agagtttgatcctggctcaggatgaacgctgacagaatgcttaacacatgcaagtatacttgatccttcgggtgatggtggcggacgggtgagtaacgcgtaaagaacttgccctgcagtctgggacaacatttggaaacgaatgctaatcccgcataagcccacagctcggcatcgagcagagggaaaaggagtgatctgctttgagatggcctcgcgtccgattagctggttggtgaggtgacggcccatcaaggcaacgatcggtagccggactgagaggttgaacggccacattgggattgagacacggcccttactcctacgggaggcagcagtggggaatattggacaatggaccaaaagtctgatccagcaattctgtgtgcacgatgaagtttttcggaatgtaaagtgctttcagttgggacgaagtaagtgacggtaccaacagaagaagcgacggctaaatacgtgccagcagccgcggtaatacgtatgtcgcaagcgttatccggatttattgggcgtaaagcgcgtctaggcggtttggtaagtctgatgtgaaaatgcggggctcaactccgtattgcgttggaaactgccaaactagagtactggagaggtgggcggaactacaagtgtagaggtgaaattcgtagatatttgtaggaatgccgatggggaagccagcccactggacagatactgacgctaaagcgcgaaagcgtgggtagcaaacaggattagataccctggtagtccacgccgtaaacgatgattactaggtgttgggggtcgaacctcagcgcccaagctaacgcgataagtaatccgcctggggagtacgtacgcaagtatgaaactcaaaggaattgacggggacccgcacaagcggtggagcatgtggtttaattcgacgcaacgcgaggaaccttaccagcgtttgacatcctaagaaattagcagagatgcttttgtgccccttcgggggaacttagtgacaggtggtgcatggctgtcgtcagctcgtgtcgtgagatgttgggttaagtcccgcaacgagcgcaacccctttcgtatgttgccatcattaagttgggcactcatgcgatactgcctgcgatgagcaggaggaaggtggggatgacgtcaagtcatcatgccccttatacgctgggctacacacgtgctacaatgggtagtacagagagtcgcaaacctgcgagggggagctaatctcagaaaactattctcagttcggattgtactctgcaactcgagtacatgaagttggaatcgctagtaatcgcaaatcagctatgttgcggtgaatacgttctcgggtcttgtacacaccgcccgt

SEQ ID NO: 38 - DNA, 1324 bp, Intestinibacter sp.; identical to SEQ ID NO: 28
  source 1..1324: mol_type = genomic DNA

SEQ ID NO: 39 - DNA, 1657 bp, Helicobacter sp.; identical to SEQ ID NO: 8
  source 1..1657: mol_type = genomic DNA

SEQ ID NO: 40 - DNA, 253 bp, Anaerobiospirillum sp.; identical to SEQ ID NO: 11
  source 1..253: mol_type = genomic DNA

SEQ ID NO: 41 - DNA, 1342 bp, Corynebacterium sp.; identical to SEQ ID NO: 29
  source 1..1342: mol_type = genomic DNA

SEQ ID NO: 42 - DNA, 1357 bp, Collinsella sp.; identical to SEQ ID NO: 12
  modified_base 766: mod_base = OTHER; note = a, c, t, g, unknown or other
  source 1..1357: mol_type = genomic DNA

SEQ ID NO: 43 - DNA, 1488 bp, Sarcina sp.
  source 1..1488: mol_type = genomic DNA
agagtttgatcctggctcaggacgaacgctggcggcgtgcctaatacatgcaagtcgagcggagttactttgagagcttgctttcaaagtaacttagcggcggacgggtgagtaacacgtaggcaacctgccccttagactgggataactaccggaaacggtagctaataccggataatttcttttttctcctgaaggaagaatgaaagacggagcaatctgtcactgagggatgggcctgcggcgcattagctagttggtggggtaacggcccaccaaggcgacgatgcgtagccgacctgagagggtgatcggccacattggaactgagatacggtccagactcctacgggaggcagcagtggggaatattgcacaatgggggaaaccctgatgcagcaacgccgcgtgagtgatgaaggtcttcggattgtaaagctctgtctttagggacgataatgacggtacctaaggaggaagccacggctaactacgtgccagcagccgcggtaatacgtaggtggcaagcgttatccggatttactgggcgtaaagggagcgtaggcggatatttaagtgggatgtgaaatacccgagcttaacttgggagctgcattccaaactggatatctagagtgcaggagaggagaatggaattcctagtgtagcggtgaaatgcgtagagattaggaagaacaccagtggcgaaggcgattctctggactgtaactgacgctgaggctcgaaagcgtggggagcaaacaggattagataccctggtagtccacgccgtaaacgatgaataccaggtgtaggggccccaagcctctgtgccgccgctaacgcattaagtattccgcctggggagtacggtcgcaagattaaaactcaaaggaattgacggggacccgcacaagcagcggagcatgtggtttaattcgaagcaacgcgaagaaccttacctagacttgacatgtcctgaattaccagtaatgtgggaagttccttcgggaacaggaacacaggtggtgcatggttgtcgtcagctcgtgtcgtgagatgttgggttaagtcccgcaacgagcgcaacccttattgttagttggtaccattaagttgaccactctagcgagactgcccgggttaaccgggaggaaggtggggatgacgtcaaatcatcatgccccttatgtctagggctacacacgtgctacaatggcaagtacaaagagaagcaatactgtgaagtggagcaaaactcaaaaacttgtctcagttcggattgtaggctgaaactcgcctacatgaagctggagttgctagtaatcgcgaatcagaatgtcgcggtgaatacgttcccgggtcttgtacacaccgcccgtcacaccatgagagttggcaatacccgaagtccgtaagctaaccgtaaggaggcagcggccgaaggtagggtcagcgattggggtgaagtcgtaacaaggtaaccaa

SEQ ID NO: 44 - DNA, 1454 bp, Clostridium sp.; identical to SEQ ID NO: 13
  modified_base 635: mod_base = OTHER; note = a, c, t, g, unknown or other
  modified_base 704: mod_base = OTHER; note = a, c, t, g, unknown or other
  source 1..1454: mol_type = genomic DNA

SEQ ID NO: 45 - DNA, 253 bp, Clostridium sp.; identical to SEQ ID NO: 14
  source 1..253: mol_type = genomic DNA

SEQ ID NO: 46 - DNA, 1392 bp, Clostridium sp.
  modified_base 811: mod_base = OTHER; note = a, c, t, g, unknown or other
  modified_base 831..832: mod_base = OTHER; note = a, c, t, g, unknown or other
  modified_base 836: mod_base = OTHER; note = a, c, t, g, unknown or other
  modified_base 999: mod_base = OTHER; note = a, c, t, g, unknown or other
  modified_base 1013: mod_base = OTHER; note = a, c, t, g, unknown or other
  modified_base 1047: mod_base = OTHER; note = a, c, t, g, unknown or other
  modified_base 1051: mod_base = OTHER; note = a, c, t, g, unknown or other
  modified_base 1057: mod_base = OTHER; note = a, c, t, g, unknown or other
  modified_base 1069: mod_base = OTHER; note = a, c, t, g, unknown or other
  modified_base 1101: mod_base = OTHER; note = a, c, t, g, unknown or other
  modified_base 1103: mod_base = OTHER; note = a, c, t, g, unknown or other
  modified_base 1116: mod_base = OTHER; note = a, c, t, g, unknown or other
  modified_base 1168: mod_base = OTHER; note = a, c, t, g, unknown or other
  modified_base 1185: mod_base = OTHER; note = a, c, t, g, unknown or other
  modified_base 1188: mod_base = OTHER; note = a, c, t, g, unknown or other
  modified_base 1202: mod_base = OTHER; note = a, c, t, g, unknown or other
  modified_base 1207: mod_base = OTHER; note = a, c, t, g, unknown or other
  modified_base 1209..1210: mod_base = OTHER; note = a, c, t, g, unknown or other
  modified_base 1221: mod_base = OTHER; note = a, c, t, g, unknown or other
  modified_base 1230: mod_base = OTHER; note = a, c, t, g, unknown or other
  modified_base 1284: mod_base = OTHER; note = a, c, t, g, unknown or other
  modified_base 1287: mod_base = OTHER; note = a, c, t, g, unknown or other
  modified_base 1296: mod_base = OTHER; note = a, c, t, g, unknown or other
  modified_base 1391: mod_base = OTHER; note = a, c, t, g, unknown or other
  source 1..1392: mol_type = genomic DNA
gggaatctccaggatctgattagcggcggacgggtgagtacacgtgggtaacctgcctcatagagtggaatagccttccgaaaggaagattaataccgcataacgttgaaagatggcatcatcattcaaccaaaggagcaatccgctatgagatggacccgcggcgcattagctagttggtggggtaacggcctaccaaggcgacgatgcgtagccgacctgagagggtgatcggccacattgggactgagacacggcccagactcctacgggaggcagcagtggggaatattgcacaatgggggaaaccctgatgcagcaacgccgcgtgagtgatgaaggttttcggatcgtaaagctctgtctttggggaagataatgacggtacccaaggaggaagccacggctaactacgtgccagcagccgcggtaatacgtaggtggcgagcgttatccggatttactgggcgtaaagggagcgtaggcggatgattaagtgggatgtgaaatacccgggctcaacttgggtgctgcattccaaactggttatctagagtgcaggagaggagagtggaattcctagtgtagcggtgaaatgcgtagagattaggaagaacaccagtggcgaaggcgactctctggactgtaactgacgctgaggctcgaaagcgtggggagcaaacaggattagataccctggtagtccacgccgtaaacgatgaatactaggtgtgggggtttcaacacctccgtgccgccgctaacgcattaagtattccgcctggggagtacggtcgcaagattaaaactnaaaggaattgacggggatcnncacnagtagcggagcatgtggtttaattcgaagcaacgcgaagaaccttacctacacttgacatcccttgcattactcttaatcgaggaaatctcttcggggacaaggtgacaggtggtgcatggttgtcgtcagctcgtgtcgtgagatgttgggttaagtcccgnaacgaggggaaccnttgtcgttagttactaccattaagttgaggactntagngagacngctgggttaacnaggaggaaggtggggatgactcaatctctggncnttatgtgtagggntacacacgtgctacaatggctggtacagagagatgcataccgggaggtggantcaatttaaaaacagtntcnttcggattgtaggntgaantnncctactgaagntggagttantagtaatcgcgaatcagaatgtcgcggtgaatacgttcccgggtcttgtacacnccncccgtcacnccatgagagttggcaatacccgaagtccgtgagctaaccgcaaggaggcagcggccgaaggtagggtcagcgattggggtgaagtcgtaacaggna

SEQ ID NO: 47 - DNA, 1362 bp, Faecalitalea sp.
  source 1..1362: mol_type = genomic DNA
gatgaacgctggcggcatgcctaatacatgcaagtcgaacggagcgaatatggaagcttgcttccgtaagagctcagtggcgaacgggtgagtaacacgtaggtaacctgcccatgtgcccgggataactgctggaaacggtagctaaaaccggataggtgaataggaggcatctcttattcattaaaggacctgtaagggtgcgaacatggatggacctgcggcgcattagctggttggagtggtaacggcacaccaaggcgacgatgcgtagccgacctgagagggcgaacggccacattgggactgagacacggcccaaactcctacgggaggcagcagtagggaattttcgtcaatggggggaaccctgaacgagcaatgccgcgtgagtgaagaaggtcttcggatcgtaaagctctgttgtaagtgaagaacggtcagtagaggaaatgatactgaagtgacggtagcttaccagaaagccacggctaactacgtgccagcagccgcggtaatacgtaggtggcgagcgttatccggaatcattgggcgtaaagggtgcgcaggtggtacattaagtccgaagtaaaaggcagcagctcaactgctgttggctttggaaactggtgaactggagtgcaggagagggcgatggaattccatgtgtagcggtaaaatgcgtagatatatggaggaacaccagtggcgaaggcggtcgcctggcctgcaactgacactgaggcacgaaagcgtggggagcaaataggattagataccctagtagtccacgccgtaaacgatgagaactaagtgttggggagactcagtgctgcagttaacgcaataagttctccgcctggggagtatgcacgcaagtgtgaaactcaaaggaattgacgggggcccgcacaagcggtggagtatgtggtttaattcgaagcaacgcgaagaaccttaccaggccttgacatggatgtaaatgttctagagatagaaagatagctatacatcacacaggtggtgcatggttgtcgtcagctcgtgtcgtgagatgttgggttaagtcccgcaacgagcgcaacccttatcgcatgttaccagtattgagttagggactcatgcgagactgccggtgacaaaccggaggaaggtggggatgacgtcaaatcatcatgccccttatggcctgggctacacacgtactacaatggcggctacaaagagaagcgaacctgcgagggggagcggaactcataaaggccgtctcagttcggattggagtctgcaactcgactccatgaagtcggaatcgctagtaatcgcagatcagcatgctgcggtgaatacgttctcgggcct

SEQ ID NO: 48 - DNA, 1399 bp, Enterococcus durans; identical to SEQ ID NO: 31
  source 1..1399: mol_type = genomic DNA

SEQ ID NO: 49 - DNA, 1414 bp, Streptococcus sp.
  source 1..1414: mol_type = genomic DNA
agagtttgatcctggctcaggactaacgctggcggcgtgcctaatacatgcaagtagaacgctgaagactttagcttgctaaagttggaagagttgcgaacgggtgagtaacgcgtaggtaacctgcctactagcgggggataactattggaaacgatagctaataccgcataacagcatttaacccatgttagatgcttgaaaggagcaattgcttcactagtagatggacctgcgttgtattagctagttggtgaggtaacggctcaccaaggcgacgatacatagccgacctgagagggtgatcggccacactgggactgagacacggcccagactcctacgggaggcagcagtagggaatcttcggcaatgggggcaaccctgaccgagcaacgccgcgtgagtgaagaaggttttcggatcgtaaagctctgttgtaagagaagaacgtgtgtgagagtggaaagttcacacagtgacggtaacttaccagaaagggacggctaactacgtgccagcagccgcggtaatacgtaggtcccgagcgttgtccggatttattgggcgtaaagcgagcgcaggcggtttaataagtctgaagttaaaggcagtggcttaaccattgttcgctttggaaactgttagacttgagtgcagaaggggagagtggaattccatgtgtagcggtgaaatgcgtagatatatggaggaacaccggtggcgaaagcggctctctggtctgtaactgacgctgaggctcgaaagcgtggggagcaaacaggattagataccctggtagtccacgccgtaaacgatgagtgaaaggtgttaggccctttccggggcttagttgctgcacgctaactgcattatgacactccgccaggggagtacgaccgctaggttgaaactcaaaggagttgacgggggccagcacaaccggtggagcatgtggttgaattggaagcaacgcgaagagccttaccaggtcttgacatcccgacgctattcctagagataggaagtttcttcgggacattcggtggcaggtggtgcatggtagtcgtcagctcgtgtcgtgagatgttgggttaagtcccgcaacgagcgcaacccctattgttagttgccatacattaagttgggcactctagcgagactgccggtaataaaccggaggaaggtggggatgacgtcaaatcatcatgccccttatgacctgggctacacacgacgctacaatggttggtacaacgagtcgcgagtcggtgacggcaagcaaatctcttaaagccaatctcagttcggattgtaggctgcaactcgcctacatgaagtcggaatcgctagtaatcgcggatcagcacgccgcggtgaatacgttcccgggccttgcactcaccgcccgtca

SEQ ID NO: 50 - DNA, 1517 bp, Streptococcus sp.
  source 1..1517: mol_type = genomic DNA
agagtttgatcatggctcaggacgaacgccggcggcgtgcctaatacatgcaagtagaacgctgaagactttagcttgctaaagttggaagagttgcgaacgggtgagtaacgcgtaggtaacctgcctactagcgggggataactattggaaacgatagctaataccgtataacagcatttaacacatgttagatgcttgaaaggagcaattgcttcactagtagatggacctgcgttgtattagctagttggtgaggtaacggctcaccaaggcgacgatacatagccgacctgagagggtgatcggccacactgggactgagacacggcccagactcctacgggaggcagcagtagggaatcttcggcaatgggggcaaccctgaccgagcaacgccgcgtgagtgaagaaggttttcggatcgtaaagctctgttgtaagagaagaacgtgtgtgagagtggaaagttcacacagtgacggtaacttaccagaaagggacggctaactacgtgccagcagccgcggtaatacgtaggtcccgagcgttgtccggatttattgggcgtaaagcgagcgcaggcggtttaataagtctgaagttaaaggcagtggcttaaccattgttcgctttggaaactgttagacttgagtgcagaaggggagagtggaattccatgtgtagcggtgaaatgcgtagatatatggarggaaacaccggtggcgaaagcggctctctggtctgtaactgacgctgaggctcgagaagcgtggggagcaaacaggattagataccctggtagtccacgccgtaagcgatgagtgctaggtgttaggccctttccggggcttagtgccgcagctaacgcattaagcactccgcctggggagtacgaccgcaaggttgaaactcaaaggaattgacgggggcccgcacaagcggtggagcatgtggtttaattcgaagcaacgcgaagaaccttaccaggtcttgacatcccgatgctattcctagagataggaagtttcttcggaacatcggtgacaggtggtgcatggttgtcgtcagctcgtgtcgtgagatgttgggttaagtcccgcaacgagcgcaacccctattgttagttgccatcattaagttgggcactctagcgagactgccggtaataaaccggaggaaggtggggatgacgtcaaatcatcatgccccttatgacctgggctacacacgtgctacaatggcggtcaacagagggaagcaatactgtgaagtggagcaaacccctaaaagccgtcccagttcggattgcaggctgcaacccgcctgtatgaagttggaatcgctagtaatcgcggatcagcatgccgcggtgaatacgttcccgggccttgtacacaccgcccgtcacaccatgagagtcgggaacacccgaagtccgtagcctaactttcacgagggggcgcggccgaaggtgggttcgataattggggtgaagtcgtaacaaggtaaccgta

SEQ ID NO: 51 - DNA, 252 bp, Streptococcus sp.
  source 1..252: mol_type = genomic DNA
tacgtaggtcccgagcgttgtccggatttattgggcgtaaagcgagcgcaggcggtttaataagtctgaagttaaaggcagtggcttaaccatttttcgctttggaaactgttagacttgagtgcagaaggggagagtggaattccatgtgtagcggtgaaatgcgtagatatatggaggaacaccggtggcgaaagcggctctctggtctgtaactgacgctgaggctcgaaagcgtggggagcaaacagg

SEQ ID NO: 52 - DNA, 1529 bp, Streptococcus sp.
  source 1..1529: mol_type = genomic DNA
agagtttgatcctggctcaggacgaacgctggcggcgtgcctaatacatgcaagtagaacgctgaagaaaggagcttgcttcttttggatgagttgcgaacgggtgagtaacgcgtaggtaacctgccttgtagcgggggataactattggaaacgatagctaataccgcataacagcttttgacacatgttagaagcttgaaagatgcaattgcatcactacgagatggacctgcgttgtattagctagtaggtagggtaacggcctacctaggcgacgatacatagccgacctgagagggtgatcggccacactgggactgagacacggcccagactcctacgggaggcagcagtagggaatcttcggcaatgggggcaaccctgaccgagcaacgccgcgtgagtgaagaaggttttcggatcgtaaagctctgttgtaagagaagaacgtgtgtgagagtggaaagttcacacagtgacggtaacttaccagaaagggacggctaactacgtgccagcagccgcggtgatacgtaggtcccgagcgttgtccggatttattgggcgtaaagcgagcgcaggcggtttaataagtctgaagttaaaggcagtggcttaaccattgttcgctttggaaactgttaaacttgagtgcagaaggggagagtggaattccatgtgtagcggtgaaatgcgtagatatatggaggaacaccggtggcgaaagcggctctctggtctgtaactgacgctgaggctcgaaagcgtggggagcaaacaggattagataccctggtagtccacgccgtaaacgatgagtgctaggtgttaggccctttccggggcttagtgccgcagctaacgcattaagtattccgcctggggagtacggtcgcaagattaaaactcaaaggaattgacgggggcccgcacaagcagcggagcatgtggtttaattcgaagcaacgcgaagaaccttacctagacttgacatctcctgcattactcttaatcgaggaagtcccttcggggacaggatgacaggtggtgcatggttgtcgtcagctcgtgtcgtgagatgttgggttaagtcccgcaacgagcgcaacccttattgttagttgccatcattaagttgggcactctagcgagactgcccgggttaaccgggaggaaggtggggatgacgtcaaatcatcatgccccttatgtctagggctacacacgtgctacaatggtcggtacaataagacgcaagcccgcgagggggagcaaaactggaaaaccgatctcagttcggattgtaggctgaaactcgcctacatgaagctggagttgctagtaatcgcgaatcagcatgtcgcggtgaatacgttcccgggccttgtacacaccgcccgtcacaccatgagagttggcaatacccaaagtacgtgatctaacccgcaagggaggaagcgtcctaaggtagggtcagcgattggggtgaagtcgtaacaaggtagccgtaggagaacctgcggctg

SEQ ID NO: 53 - DNA, 1398 bp, Streptococcus sp.
  source 1..1398: mol_type = genomic DNA
agagtttgctcttgggtcaggatgaacgctggcggcgtgcttaacacatgcaagtcgagcgagaaaagttcttcggagcttttctagcggcggacgggtgagtaacacgtgggcaacctgcctcatagaggggaatagccttccgaaaggaagattaataccgcataacattgttgaaaggcatcttttaacaatcaaaggagcaatccgctatgagatgggcccgcggcgcattagctagttggtgaggtaacggctcaccaaggcgacgatgcgtagccgacctgagagggtgatcggccacattggaactgagacacggtccagactcctacgggaggcagcagtggggaatattgcacaatgggggaaaccctgatgcagcgacgccgcgtgagtgaagaagtatttcggtatgtaaagctctgttgtaagagaagaacgtgtgtgagagtggaaagttcacacagtgacggtaacttaccagagagggacggctaactacgtgccagcagccgcggtaatacgtaggtcccgagcgttgtccggatttattgggcgtaaagcgagcgcaggcggtttaataagtctgaagttaaaggcagtggcttaaccattgttcgctttggaaactgttagacttgagtgcagaaggggagagtggaattccatgtgtagcggtgaaatgcgtagatatatggaggaacaccggtggcgaaagcggctctctggtctgtaactgacgctgaggctcgaaagcgtggggagcaaacaggattagataccctggtagtccacgccgtaaacgatgagtgctaggtgttaggccctttccggggcttagtgccgcagctaacgcattaagcactccgcctggggagtacgaccgcaaggttgaaactcaaaggaattgacgggggcccgcacaagcggtggagcatgtggtttaattcgaagcaacgcgaagaaccttaccaggtcttgacatcccgatgctattcctagagataggaagtttcttcggaacatcggtgacaggtggtgcatggttgtcgtcagctcgtgtcgtgagatgttgggttaagtcccgcaacgagcgcaacccctattgttagttgccatcattaagttgggcactctagcgagactgccggtaataaaccggaggaaggtggggatgacgtcaaatcatcatgccccttatgacctgggctacacacgtgctacaatggttggtacaacgagtcgcgagtcggtgacggcaagcaaatctcttaaagccaatctcagttcggattgtaggctgcaactcgcctacatgaagtcggaatcgctagtaatcgcggatcagcacgccgcggtgaatacgttcccgggccttgcactcaccgcccgtca

SEQ ID NO: 54 - DNA, 1393 bp, Streptococcus sp.; identical to SEQ ID NO: 32
  modified_base 1381: mod_base = OTHER; note = a, c, t, g, unknown or other
  source 1..1393: mol_type = genomic DNA

SEQ ID NO: 55 - DNA, 1456 bp, Streptococcus sp.
  source 1..1456: mol_type = genomic DNA
ttcaggacgaacgctggcggcgtgcctaatacatgcaagtagaacgctgaagactttagcttgctaaagttggaagagttgcgaacgggtgagtaacgcgtaggtaacctgcctactagcgggggataactattggaaacgatagctaataccgcataacagcatttaacccatgttagatgcttgaaaggagcaattgcttcactagtagatggacctgcgttgtattagctagttggtgaggtaacggctcaccaaggcgacgatacatagccgacctgagagggtgatcggccacactgggactgagacacggcccagactcctacgggaggcagcagtagggaatcttcggcaatgggggcaaccctgaccgagcaacgccgcgtgagtgaagaaggttttcggatcgtaaagctctgttgtaagagaagaacgtgtgtgagagtggaaagttcacacagtgacggtaacttaccagaaagggacggctaactacgtgccagcagccgcggtaatacgtaggtcccgagcgttgtccggatttattgggcgtaaagcgagcgcaggcggtttaataagtctgaagttaaaggcagtggcttaaccattgttcgctttggaaactgttagacttgagtgcagaaggggagagtggaattccatgtgtagcggtgaaatgcgtagatatatggaggaacaccggtggcgaaagcggctctctggtctgtaactgacgctgaggctcgaaagcgtggggagcaaacaggattagataccctggtagtccacgccgtaaacgatgagtgctaggtgttaggccctttccggggcttagtgccgcagctaacgcattaagcactccgcctggggagtacgaccgcaaggttgaaactcaaaggaattgacgggggcccgcacaagcggtggagcatgtggtttaattcgaagcaacgcgaagaaccttaccaggtcttgacatcctttgaccactctagagatagagcttccccttcgggggcaaagtgacaggtggtgcatggttgtcgtcagctcgtgtcgtgagatgttgggttaagtcccgcaacgagcgcaacccttattgttagttgccatcatttagttgggcactctagcgagactgccggtgacaaaccggaggaaggtggggatgacgtcaaatcatcatgccccttatgacctgggctacacacgtgctacaatgggaagtacaacgagttgcgaagtcgcgaggctaagctaatctcttaaagcttctctcagttcggattgtaggctgcaactcgcctacatgaagccggaatcgctagtaatcgcggatcagcacgccgcggtgaatacgttcccgggccttgtacacaccgcccgtcacaccacgagagtttgtaacacccgaagtcggtgaggtaaccttttaggagccagccgcctaagg

SEQ ID NO: 56 - DNA, 1442 bp, Streptococcus sp.
  source 1..1442: mol_type = genomic DNA
ctaatacatgcgaggagaacgctgaagactttcttttgctatagttgggagagttgctaacgggtgagtaacgcgtaggtgacctgcctactagcgggggataactattgcaaacgatagctaataccgcataacagcctttaacccatgttagatgcttgaaaggagcaattgcttcactagtagatggacctgcgttgtattagctagttggtgaggtaacggctcaccaaggcgacgatacatagccgacctgagagggtgatcggccacactgggactgagacacggcccatactcctacgggaggcaccagtagggaatcttcgggaatgggggcaaccctgaccgagcaacgccgcgtgagtgaagaaggttttcggatcgtaaagctctgttgtaagagaagaacgtgtgtgagagtggaaagttcacactgtgacggtaacttaccagaaagggacggctaactacgtgccagcagccgcggtaatacgtaggtcccgagcgttgtccggatttattgggcgtaaagcgagcgcaggcggtttaataagtctgaagttaaaggcagtggcttaaccattgttcgctttggaaactgttagacttgagtgcataaggggagagtggaattccatgtgtagcggtgaaatgcgtagatatatggaggaacaccggtggcgaaagcggctctctggtctgtaactgacgttgaggctcgaaagcgtggggagcaaacaggattagataccctggtagtccacgctgtaaacgatgagtggtaggtgttaggccctttctggggtttagtgccgcagattacgcattaagccattcgcctggggagtacgaccgcaaggttgaaacttaaaggaattgacgggggcccgcacaagcggtggagcatgtggtttaattagaagcaacgcgaagaaccttaccaggtcttgacatcccgatgctattcttagagataggaagtttcttcggaacatcggtgacaggtggtgcatggttgtcgtcagctcgtgtcgagagatgttgggttaagtccctcaacgagcgcaacccctatttttatttgccatcattaagttgggcaatctagcgagactgccggtaataaaccggaggaaggtggggatgacgtcaaatcatcatgctccttatgtcatggggtacacacgtggtacaatggttggtacaacgagtcgcgagttggtgaaggcaagcaaatctcttaaagccaatatcagttcggattgtaggctgcaaatagcctacatgtagtcggaattgttagtaatcggggatcagcactccgcggtgaatacgtttccgggccttgtacaccccgcccgtctacaccacgagagtttgtaacacccgaagtcggtgaggtaactcttttaggagccagccgcctaaggtgggataga

SEQ ID NO: 57 - DNA, 1382 bp, Erysipelatoclostridium sp.
  source 1..1382: mol_type = genomic DNA
agagtttgattatggctcaggatgaacgctggcggcgtgcctaatacatgcaagtcgaacgcgagcagcaatgctcgagtggcgaacgggtgagtaatacataagtaacctgccctagacagggggataactgctggaaacggcagctaagaccgcataggtatggacactgcatggtgaccatattaaaagtgccaaggcactggtagaggatggacttatggcgcattagctggttggtgaggtaacggctcaccaaggcgacgatgcgtagccgacctgagagggtgaccggccacactgggactgagacacggcccagactcctacgggaggcagcagtagggaattttcggcaatggggggaaccctgaccgagcaacgccgcgtgaaggaagaaggaattcgttctgtaaacttctgttataaaggaagaacggcggatatagggaatgatatccgagtgacggtactttatgagaaagccacggctaactacgtgccagcagccgcggtaatacgtaggtggcgagcgttatccggaattattgggcgtaaagagggagcaggcggcggcagaggtctgtggtgaaagactgaagcttaacttcagtaagccatagaaaccgggctgctagagtgcaggagaggatcgtggaattccatgtgtagcggtgaaatgcgtagatatatggaggaacaccagtggcgaaggcgacggtctggcctgtaactgacgctcattcccgaaagcgtggggagcaaataggattagataccctagtagtccacgccgtaaacgatgagtactaagtgttgggagtcaaatttcagtgctgcagttaacgcaataagtactccgcctgagtagtacgttcgcaagaatgaaactcaaaggaattgacgggggcccgcacaagcggtggagcatgtggtttaattcgatgatacgcgaggaaccttaccagggcttaaatgtgactgacaggtccggaaacggacttttcttcggacagttacaggtgctgcatggttgtcgtcagctcgtgccgtgaggtgtcaggttaagtcctataacgagcgcaacccctgtcgctagttgccagcgagtaatgtcgggaactctagcgagactgccagtgcaaactgcgaggaaggtggggatgacgtcaaatcatcacggcccttacgccctgggctacacacgtgctacaatggccggtacagagagcagccaccccgcgagggggagcgaatctacaaaaccggtcacagttcggatcggagtctgcaactcgactccgtgaagctggaatcgctagtaatcggatatcagccatgatccggtgaatacgttcccgggccttgtacacacccccgtc

SEQ ID NO: 58 - DNA, 1418 bp, Megasphaera sp.; identical to SEQ ID NO: 33
  source 1..1418: mol_type = genomic DNA

SEQ ID NO: 59 - DNA, 1383 bp, unidentified
  misc_feature 1..1383: note = source = /note="Description of Unknown: Lachnospiraceae sequence"
  source 1..1383: mol_type = genomic DNA
agagtttgatcctggctcaggatgaacgctggcggcgtgcttaacacatgcaagtcgaacgggaaacttttcattgaagcttcggcagatttggtctgtttctagtggcggacgggtgagtaacgcgtgggtaacctgccttatacagggggataacaaccagaaatggttgctaataccgcataagcgcacaggaccgcatggtccggtgtgaaaaactccggtggtataagatggacccgcgttggattagctagttggcagggtaacggcctaccaaggcgacgatccatagccggcctgagagggtgaacggccacattgggactgagacacggcccagactcctacgggaggcagcagtggggaatattgcacaatgggggaaaccctgatgcagcgacgccgcgtgaaggaagaagtatctcggtatgtaaacttctatcagcagggaagatagtgacggtacctgactaagaagccccggctaaatacgtgccagcagccgcggtaatacgtatggttcaagcgttatccggatttactgggtgtaaagggtgagtaggcggttatgcaagtcatatgtgaaatgtcggggctcaactccggcctgcataagaaactgtataactagagtgcaggagaggcaagcggaattcctagtgtagcggtgaaatgcgtagatattaggaagaacaccggtggcgaaggcggcttgctggactgttactgacgctgagtcacgaaagcgtggggagcaaacaggattagataccctggtagtccacgccgtaaacgatgaatactaggtgtcgggtggcaaagccattcggtgccgcagcaaacgcaataagtattccacctggggagtacgttcgcaagaatgaaactcaaaggaattgacggggacccgcacaagcggtggagtatgtggtttaattcgaagcaacgcgaagaaccttaccaggccttgacatggatataaatgttctagagatagaaagatagctatatatcacacaggtggtgcatggttgtcgtcagctcgtgtcgtgagatgttgggttaagtcccgcaacgagcgcaacccttgtcttctgttaccagcattgagttggggactcaggagagactgccggtgacaaaccggaggaaggtggggatgacgtcaaatcatcatgccccttatggcctgggctacacacgtactacaatggcgcctacaaagagcagcgacaccgcgaggtgaagcgaatctcataaagggcgtctcagttcggattgaagtctgcaactcgacttcatgaagtcggaatcgctagtaatcgcagatcagcatgctgcggtgaatacgttcccgggtcttgtactcaccgcccgtca

SEQ ID NO: 60 - DNA, 1361 bp, Blautia sp.
  source 1..1361: mol_type = genomic DNA
gatgaacgctggcggcgtgcttaacacatgcaagtcgagcgaagcacttaagtggatctcttcggattgaaacttatttgactgagcggcggacgggtgagtaacgcgtgggtaacctgcctcatacagggggataacagttagaaatggctgctaataccgcataagcgcacaggaccgcatggtctggtgtgaaaaactccggtggtatgagatggacccgcgtctgattagctagttggaggggtaacggcccaccaaggcgacgatcagtagccggcctgagagggtgaacggccacattgggactgagacacggcccagactcctacgggaggcagcagtggggaatattgcacaatgggggaaaccctgatgcagcgacgccgcgtgaaggaagaagtatctcggtatgtaaacttctatcagcagggaagaaaatgacggtacctgactaagaagccccggctaactacgtgccagcagccgcggtaatacgtagggggcaagcgttatccggatttactgggtgtaaagggagcgtagacggaagagcaagtctgatgtgaaaggctggggcttaaccccaggactgcattggaaactgtttttctagagtgccggagaggtaagcggaattcctagtgtagcggtgaaatgcgtagatattaggaggaacaccggtggcgaaggcggcttactggacgaccactgacgctgaggctcgaaagcgtggggagcaaacaggattagataccctggtagtccacgccgtaaaccgatgaataataggtgtcggggaacaatagttctttggtgccgcagcaaaacgcattaagtattccacctggggagtacgttcgcaagaatgaaactcaaaggaattgacggggacccgcacaagcggtggagcatgtggtttaattcgatgcaacgcgaagaaccttacctgctcttgacatcccactgaccggacagtaatgtgtccttttcttctgaacagtggagacaggtggtgcatggttgtcgtcagctcgtgtcgtgagatgttgggttaagtcccgcaacgagcgcaaccctcgtctttagtagccagcagtccggctgggcactctagagagactgccagggataacctggaggaaggcggggaggacgtcaaatcatcatgccccttacgagcagggctacacacgtgctacaatggcgtaaacaaagggaagcgaccccgtgaaggtgagcaaatctcaaaaataacgtctcagttcggattgtagtctgcaactcgactacatgaagctggaatcgctagtaatcgcgaatcagaatgtcgcggtgaataaaaggccgggtcttgcaca

SEQ ID NO: 61 - DNA, 253 bp, Alloprevotella sp.
  source 1..253: mol_type = genomic DNA
tacggaaggtccaggcgttatccggatttattgggtttaaagggagcgcaggcggactcttaagtcagttgtgaaatacggcggctcaaccgtcggactgcagttgatactgggagtcttgagtacacgcagagatactggaattcatggtgtagcggtgaaatgctcagatatcatgaggaactccgatcgcgaaggcaggtatctggagtgtaactgacgctgaggctcgaaagtgcgggtatcaaacagg

SEQ ID NO: 62 - DNA, 1394 bp, Parabacteroides sp.; identical to SEQ ID NO: 18
  source 1..1394: mol_type = genomic DNA

SEQ ID NO: 63 - DNA, 1445 bp, Bacteroides sp.
  source 1..1445: mol_type = genomic DNA
tacaggcttaacacatgcaagtcgaggggcagcatgattgaagcttgcttcaattgatggcgaccggcgcacgggtgagtaacacgtatccaaccttccgtacactcagggatagcctttcgaaagaaagattaatacctgatggtatcttaagcacacatgtaattaagattaaagatttatcggtgtacgatggggatgcgttccattaggtagtaggcggggtaacggcccacctagcctacgatggatgggggttctgagaggaaggtcccccacattggaactgagacacggtccaaactcctacgggaggcagcagtgaggaatattggtcaatggacgagagtctgaaccagccaagtagcgtgaaggatgaaggtcctacggattgtaaacttcttttataagggaataaaacctcccacgtgtgggagcttgtatgtaccttatgaataagcatcggctaactccgtgccagcagccgcggtaatacggaggatgcgagcgttatccggatttattgggtttaaagggagcgcagacgggtcgttaagtcagctgtgaaagtttggggctcaaccttaaaattgcagttgatactggcgtccttgagtgcggttgaggtgtgcggaattcgtggtgtagcggtgaaatgcttagatatcacgaagaactccgattgcgaaggcagcacactaagccgtaactgacgttcatgctcgaaagtgtgggtatcaaacaggattagataccctggtagtccacacagtaaacgatgaatactcgctgtttgcgatatacagtaagcggccaagcgaaagcattaagtattccacctggggagtacgccggcaacggtgaaactcaaaggaattgacgggggcccgcacaagcggaggaacatgtggtttaattcgatgatacgcgaggaaccttacccgggcttaaattgcatttgaatatattggaaacagtatagccgtaaggcaaatgtgaaggtgctgcatggttgtcgtcagctcgtgccgtgaggtgtcggcttaagtgccataacgagcgcaacccttatcttcagttactaacaggtcatgctgaggactctggagagactgccgtcgtaagatgtgaggaaggtggggatgacgtcaaatcagcacggcccttacgtccggggctacacacgtgttacaatggggggtacagaaggccgctacctggtgacaggatgctaatcccaaaagcctctctcagttcggatcgaagtctgcaacccgacttcgtgaagctggattcgctagtaatcgcgcatcagccatggcgcggtgaatacgttcccgggccttgtacacaccgcccgtcaagccatgaaagccgggggtacctgaagtacgtaaccgcaaggagcgtcctagggtaaaactggtaattggggctaagtcata

SEQ ID NO: 64 - DNA, 1522 bp, unidentified
  misc_feature 1..1522: note = source = /note="Description of Unknown: Escherichia-Shigella sequence"
  source 1..1522: mol_type = genomic DNA
agagtttgatcatggctcagattgaacgctggcggcaggcctaacacatgcaagtcgaacggtaacaggaagaagcttgcttctttgctgacgagtggcggacgggtgagtaatgtctgggaaactgcctgatggagggggataactactggaaacggtagctaataccgcataacgtcgcaagaccaaagagggggaccttcgggcctcttgccatcggatgtgcccagatgggattagctagtaggtggggtaacggctcacctaggcgacgatccctagctggtctgagaggatgaccagccacactggaactgagacacggtccagactcctacgggaggcagcagtggggaatattgcacaatgggcgcaagcctgatgcagccatgccgcgtgtatgaagaaggccttcgggttgtaaagtactttcagcggggaggaagggagtaaagttaatacctttgctcattgacgttacccgcagaagaagcaccggctaactccgtgccagcagccgcggtaatacggagggtgcaagcgttaatcggaattactgggcgtaaagcgcacgcaggcggtttgttaagtcagatgtgaaatccccgggctcaacctgggaactgcatctgatactggcaagcttgagtctcgtagaggggggtagaattccaggtgtagcggtgaaatgcgtagagatctggaggaataccggtggcgaaggcggccccctggacgaagactgacgctcaggtgcgaaagcgtggggagcaaacaggattagataccctggtagtccacgccgtaaacgatgtcgacttggaggttgtgcccttgaggcgtggcttccggagctaacgcgttaagtcgaccgcctggggagtacggccgcaaggttaaaactcaaatgaattgacgggggcccgcacaagcggcggagcatgtggattaattcgatgcaacgcgaagaaccttacctgggtttgacatgcacaggacgcgtctagagataggcgttcccttgtggcctgtgtgcaggtggtgcatggctgtcgtcagctcgtgtcgtgagatgttgggttaagtcccgcaacgagcgcaacccttgtctcatgttgccagcacgtaatggtggggactcgtgagagactgccggggtcaactcggaggaaggtggggatgacgtcaagtcatcatgccccttatgtccagggcttcacacatgctacaatggccggtacaaagggctgcgatgccgcgaggttaagcgaatccttaaaagccggtctcagttcggatcggggtctgcaactcgaccccgtgaagtcggagtcgctagtaatcgcagatcagcaacgctgcggtgaatacgttcccgggccttgtacacaccgcccgtcacgtcatgaaagtcggtaacacccgaagccagtggcctaaccctcgggagggagctgtcgaaggtgggatcggcgattgggacgaagtcgtaacaaggtaaccgtaggggaacctgcggttg

SEQ ID NO: 65 - DNA, 1472 bp, unidentified; identical to SEQ ID NO: 35
  misc_feature 1..1472: note = source = /note="Description of Unknown: Escherichia-Shigella sequence"
  source 1..1472: mol_type = genomic DNA

SEQ ID NO: 66 - DNA, 1374 bp, Blautia sp.
  source 1..1374: mol_type = genomic DNA
agagtttgatcatggctcaggatgaacgctagctacaggcttaacacatgcaagtcgaggggcagcatggtcttagcttgctaaggccgatggcgaccggcgcacgggtgagtaacacgtatccaacctgccgtctactcttggacagccttctgaaaggaagattaatacaagatggcatcatgagtccgcatgttcacatgattaaaggtattccggtagacgatggggatgcgttccattagatagtaggcggggtaacggcccacctagtcttcgatgggtaggggttctgagaggaaggtcccccacattggaactgagacacggcccaaactcatacgggaggcagcagtggggaatattgcacaatgggggaaaccctgatgcagcgacgccgcgtgaaggatgaagtatttcggtatgtaaacttctatcagcagggaagaaaatgacggtacctgactaagaagccccggctaactacgtgccagcagccgcggtaatacgtagggggcaagcgttatccggatttactgggtgtaaagggagcgtagacggcagtgcaagtctgaagtgaaagcccggggctcaaccccgggactgctttggaaactgtgcagctagagtgtcggagaggcaagcggaattcctagtgtagcggtgaaatgcgtagatattaggaggaacaccagtggcgaaggcggcttgctggacgatgactgacgttgaggctcgaaagcgtggggagcaaacaggattagataccctggtagtccacgccgtaaacgatgactactaggtgtcggggagcaaagctcttcggtgccgcagccaacgcaataagtagtccacctggggagtacgttcgcaagaatgaaactcaaaggaattgacggggacccgcacaagcggtggagcatgtggtttaattcgaagcaacgcgaagaaccttacctgctcttgacatccctctgaccgctctttaatcggagctttccttcgggacagaggagacaggtggtgcatggttgtcgtcagctcgtgtcgtgagatgttgggttaagtcccgcaacgagcgcaacccttatggtcagttactacgcaagaggactctggccagactgccgttgacaaaacggaggaaggtggggatgacgtcaaatcatcatgccctttatgacttgggctacacacgtactacaatggcgttaaacaaagagaagcgagaccgcgaggtggagcaaaactcggaaacaacgtcccagttcggactgcaggctgcaactcgcctgcacgaagtcggaattgctagtaatcgcagatcagcatgctgcggtgaatacgttcccgggccttgcactcaccgcccgt

SEQ ID NO: 67 - DNA, 1440 bp, Tyzzerella sp.; identical to SEQ ID NO: 36
  source 1..1440: mol_type = genomic DNA

SEQ ID NO: 68 - DNA, 1370 bp, Ruminococcus gauvreauii
  source 1..1370: mol_type = genomic DNA
atgaacgctggcggcgtgcctaacacatgcaagtcgaacgaagcgcttgaacggatatcttcggactgaagttcttgcgactgagtggcggacgggtgagtaacgcgtgggtaacctgcctcatacagggggataacagttagaaatgactgctaataccgcataagcgcacagcttcgcatggagcagtgtgaaaaactccggtggtatgagatggacccgcgtcagattagctagttggcagggtaacggcctaccaaggcgacgatctgtagccgacctgagagggtgaccggccacattgggactgagacacggcccaaactcctacgggaggcagcagtggggaatattgcacaatgggggaaaccctgatgcagcgacgccgcgtgagcgaagaagtatttcggtatgtaaagctctatcagcagggaagataatgacggtacctgactaagaagctccggctaaatacgtgccagcagccgcggtaatacgtatggagcaagcgttatccggatttactgggtgtaaagggagcgtagacggtttgacaagtctgatgtgaaattccagggcttaaccctggacctgcattggaaactgtcggactagagtgtcggagaggtgagtggaattcctagtgtagcggtgaaatgcgtagatattaggaggaacaccagtggcgaaggcggctcactggacgataactgacgttgaggctcgaaagcgtggggagcaaacaggattagataccctggtagtccacgccgtaaacgatgtgtactaggtgttggggagcaaagctcttcggtgccgtcgcaaacgcagtaagtacaccacctggggagtacgttcgcaagaatgaaactcaaaggaattgacggggacccgcacaagcggtggagcatgtggtttaattcgaagcaacgcgaagaaccttaccaaatcttgacatcggagtgaccgctctttaatcggagctttccttcgggacactccagacaggtggtgcatggttgtcgtcagctcgtgtcgtgagatgttgggttaagtcccgcaacgagcgcaacccttatccttagtagccagcaagtgaagttgggcactctagggagactgccagggataacctggaggaaggtggggatgacgtcaaatcatcatgccccttatgatttgggctacacacgtgctacaatggcgtaaacaaagggaagcgatcacgtgagtgtgagcaaatctcaaaaataacgtcccagttcggactgtagtctgcaacccgactacacgaagctggaatcgctagtaatcgcaggtcagcatactgcggtgaatacgttcccgggtcttgcacacaccgcccgtca

SEQ ID NO: 69 - DNA, 1366 bp, Fusobacterium sp.; identical to SEQ ID NO: 37
  source 1..1366: mol_type = genomic DNA

SEQ ID NO: 70 - DNA, 1361 bp, Fusobacterium sp.
  source 1..1361: mol_type = genomic DNA
agagtttgatcctggctcaggacgaacgctggcggcgtgcctaacacatgcaagtcgagcgattctcttcggagaagagcggcggacgggtgagtaacgcgtgggtaacctgccctgtacacacggataacataccgaaaggtatgctaatacgggataatatataagagtcgcatgacttttatatcaaagatttttcggtacaggatggacccgcgtctgattagcttgttggcggggtaacggcccaccaaggcgacgatcagtagccgacctgagagggtgatcggccacattggaactgagacacggtccaaactcctacgggaggcagcagtggggaatattgcacaatgggcgcaagcctgatgcagcaacgccgcgtgagcgatgaaggccttcgggtcgtaaagctctgtcctcaaggaagataatgacggtacttgaggaggaagccccggctaactacatgccagcagccgcggtaatacgtatgtcgcaagcgttatccggatttattgggcgtaaagcgcgtctaggtggtttggtaagtctgatgtgaaaatgcggggctcaactccgtattgcgttggaaactgccaaactagagtactggagaggtaggcggaactacaagtgtagaggtgaaattcgtagatatttgtaggaatgccgatggggaagccagcctactggacagatactgacgctaaagcgcgaaagcgtgggtagcaaacaggattagataccctggtagtccacgccgtaaacgatgattactaggtgttgggggtcgaacctcagcgcccaagctaacgcgataagtaatccgcctggggagtacgtacgcaagtatgaaactcaaaggagttgacggggacccgcacaagcggtggagcatgtggtttaattcgacgcaacgcgaggaaccttaccagcgtttgacatcctaggaatgagaaagagatttcttagtgctccttcgggagaacctagagacaggtggtgcatggctgtcgtcagctcgtgtcgtgagatgttgggttaagtcccgcaacgagcgcaacccctattgtatgttgccatcattaagttgggcactcatgcgatactgcctgcgatgagcaggaggaaggtggggatgacgtcaagtcatcatgccccttatacgctgggctacacacgtgctacaatgggcagtacagagagaagcaataccgcgaggtggagccaaacttaaaaaccagtctcagttcggattgtaggctgaaactcgcctacatgaagctggagttactagtaatcgcgaatcagaatgtcgcggtgaatacgtacccgggtcttgtacacaccgcccgtca

SEQ ID NO: 71 - DNA, 1360 bp, unidentified
  misc_feature 1..1360: note = source = /note="Description of Unknown: Lachnospiraceae sequence"
  source 1..1360: mol_type = genomic DNA
gatgaacccttgcggcgtgcttaacacatgcaagtcgaacgggaaacattttattgaagcttcggcagatctagcttgtttctagtggcggacgggtgagtaacgcgtgggcaacctgcctcacactgggggataacagtcagaaatggctgctaataccgcataagcgcacagcatcgcatgatgcagtgtgaaaaactccggtggtgtgagatggacccgcgttggattagctagttggcagggcagcggcctaccaaggcgacgatccatagccggcctgagagggtgaacggccacattgggactgagacacggcccagactcccacgggaggcagcagtggggaatattgcacaatgggggaaaccctgatgcagcgacgccgcgtgaaggaagaagtatctcggtatgtaaacttctatcagcagggaagaaaatgacggtacctgactaagaagccccggctaactacgtgccagcagccgcggtaatacgtagggggcaagcgttatccggatttactgggtgtaaagggagcgtagacggtgttgcaagtctgatgtgaaaggcgggggctcaacccctggactgcattggaaactgtgatactcgagtgccggagaggtaagcggaattcctagtgtagcggtgaaatgcgtagatattagaaggaataccagtggcgaaggcggcttactggacggtaactgacgttgaggctcgaaagcgtggggagcaaacaagattaagaaacctctgggtagtccacgcccgtaaacgaaggaataaaggggtcgggagcagagcttttcggtgccgcagcaaacccaataagtattccaccttgagaggacgttcgcaagaatgaaactcaaaggaattgacgggggacccgcacaagcggtggagcatgtggtttaattcgaagcaacgcgaagaaccttaccaagtcttgacatccctctgaccgcaccttaaccggtgctttccttcgggacagaggagacaggtggtgcatggttgtcgtcagctcgtgtcgtgagatgttgggttaagtcccgcaacgagcgcaacccttatccttagtagccagcggtccggccgggcactctggggagactgccagggataacctggaggaaggtggggatgacgtcaaatcatcatgccccttatgatttgggctacacacgtgctacaatggcgtaaacaaagggaagcgatcacgtgagtgcgagcaaatctcaaaaataacgtcccagttcggactgtagtctgcaacccgactacacgaagctggaatcgctagtaatcgcaggtcagcatactgcggtgaatacgttcccgggtcttgtac

SEQ ID NO: 72 - DNA, 1332 bp, Blautia sp.; identical to SEQ ID NO: 26
  source 1..1332: mol_type = genomic DNA

SEQ ID NO: 73 - DNA, 1311 bp, unidentified
  modified_base 725: mod_base = OTHER; note = a, c, t, g, unknown or other
  modified_base 727: mod_base = OTHER; note = a, c, t, g, unknown or other
  modified_base 740: mod_base = OTHER; note = a, c, t, g, unknown or other
  modified_base 747..748: mod_base = OTHER; note = a, c, t, g, unknown or other
  misc_feature 1..1311: note = source = /note="Description of Unknown: Peptostreptococcaceae sequence"
  source 1..1311: mol_type = genomic DNA
gatgaacgctggcggcgtgcctaacacatgcaagtcgagcgatttacttcggtaaagagcggcggacgggtgagtaacgcgtgggtaacctgccctgtacacacggataacataccgaaaggtatgctaatacgagataatatgcttttatcgcatggtagaagtatcaaagcttttgcggtacaggatggacccgcgtctgattagctagttggtaaggtaacggcttaccaaggcaacgatcagtagccgacctgagagggtgatcggccacattggaactgagacacggtccaaactcctacgggaggcagcagtggggaatattgcacaatgggcgaaagcctgatgcagcaacgccgcgtgagcgatgaaggccttcgggtcgtaaagctctgtcctcaaggaagataatgacggtacttgaggaggaagccccggctaactacgtgccagcagccgcggtaatacgtagggggctagcgttatccggaattactgggcgtaaagggtgcgtaggtggtttcttaagtcagaggtgaaaggctacggctcaaccgtagtaagcctttgaaactgggaaacttgagtgcaggagaggagagtggaattcctagtgtagcggtgaaatgcgtagatattaggaggaacaccagttgcgaaggcggctctctggactgtaactgacactgaggcacgaaagcgtgggagcaaacaagattagntnccctggtagtccncgccgtnnccgcccataaagagctgtcggaggttacccccttcggtggcgcaggtaacgcaataaagaattccgcctgggaaggaacgcttcgcaagagtgaaattaaaaggaatagacggggacccgctcaagtagtggagcatgtggtttaattcgaagcaacgcgaagaactttctctaagcttgacatccttttgaccgatgcctaatagcatcaatcccttctgggacagaagtgacaggtggtgcatggttgttgtcagctcgtgtcgtgagatgttgggttaagtcccgcaacgagcgcaacccttgcctttagttgccagcattaagttgggcactctatagggactgccagggataacctggaggaaggtggggatgacgtcaaatcatcatgccccttatgcttagggctacacacgtgctacaatgggtggtacagagggcagccaagtcgtgaggcggagctaatcccttaaagccattctcagttcggattgtaggctgaaactcgcctacatgaagctggagttactagtaatcgcagatcagaatgatgcggtgaa

SEQ ID NO: 74 - DNA, 1324 bp, Intestinibacter sp.; identical to SEQ ID NO: 28
  source 1..1324: mol_type = genomic DNA

SEQ ID NO: 75 - DNA, 1288 bp, Peptoclostridium sp.
  source 1..1288: mol_type = genomic DNA
gaaagcggcggacgggtgagtaacgcgtaggcaacctgccccatacagagggatagcatctggaaacggatattaatacctcataatacttagagatcacatggtaactaagtcaaagatttatcggtatgggatgggcctgcgtctgattagctagttggtggggtaacggctcaccaaggcgacgatcagtagccgacctgagagggtgatcggccacattggaactgagacacggtccaaactcctacgggaggcagcagtggggaatattgcacaatgggcgcaagcctgatgcagcaacgccgcgtgagcgatgaaggccttcgggtcgtaaagctctgtcctcaaggaagataatgacggtacttgaggaggaagccccggctaactacgtgccagcagccgcggtaatacgtagggggctagcgttatccggatttactgggcgtaaagggtgcgtaggcggtctttcaagtcaggagttaaaggctacggctcaaccgtagtaagctcctgatactgtctgacttgagtgcaggagaggaaagcggaattcccagtgtagcggtgaaatgcgtagatattgggaggaacaccagtagcgaaggcggctttctggactgtaactgacgctgaggcacgaaagcgtggggagcaaacaggattagataccctggtagtccacgctgtaaacgatgagtactaggtgtcggaggttacccccttcggtgccgcagctaacgcattaagtactccgcctggggagtacgcacgcaagtgtgaaactcaaaggaattgacggggacccgcacaagtagcggagcatgtggtttaattcgaagcaacgcgaagaaccttacctaggcttgacatccttctgaccgaggactaatctcctctttccctccggggacagaagtgacaggtggtgcatggttgtcgtcagctcgtgtcgtgagatgttgggttaagtcccgcaacgagcgcaacccttgtctttagttgccatcattaagttgggcactctagagagactgccagggataacctggaggaaggtggggatgacgtcaaatcatcatgccccttatgcctagggctacacacgtgctacaatgggtggtacagagggcagccaagccgtgaggtggagcaaatcccttaaagccattctcagttcggattgtaggctgaaactcgcctacatgaagctggagttactagtaatcgcagatcagaatgctgcggtgaatgcgttcccgggtcttgcacacaccgcccgtca

SEQ ID NO: 76 - DNA, 1391 bp, Sutterella sp.
  source 1..1391: mol_type = genomic DNA
ctggctcaggatgaacgctagcgacaggcttaacacatgcaagtcgaggggcatcacgggaggtagcaataccttctggtggcgaccggcgcacgggtgagtaacacgtatgcaacctgccctgtacagagggacaagcggtggaaacgccgtctaatcccgcatgcactcttccgggggcatccccgggagagtaaaggagagatccggtacaggatggacatgcggcgcattagttagttggcggggtaacggcccaccaagacgacgatgcgtaggggttctgagaggaaggtcccccacattggaactgagacacggtccaaactcctacgggaggcagcagtgaggaatattggtcaatgggcggaagcctgaaccagccaagtcgcgtgagggaagacggccctacgggttgtaaacctcttttgtcggggagcaatgccgcctttgcgaaggcggagggagagtacccgaagaaaaagcaccggctaactacgtgccagcagccgcggtaatacgtagggtgcaagcgttaatcggaattactgggcgtaaagcgtgcgcaggcggttctgtaagacagatgtgaaatccccgggctcaacctgggaattgcatttgtgactgcaggactagagttcatcagaggggggtggaattccaagtgtagcagtgaaatgcgtagatatttggaagaacaccaatggcgaaggcagccccctgggatgcgactgacgctcatgcacgaaagcgtggggagcaaacaggattagataccctggtagtccacgccctaaacgatgtctactggttgttggggattaatatccttggtaacgaagctaacgcgtgaagtagaccgcctggggagtacggtcgcaagattaaaactcaaaggaattgacggggacccgcacaagcggtggatgatgtggattaattcgatgatacgcgaggaaccttacccgggctcaaacggcacagtgatacttttgaaaggaggtagctctacggagactgtgccgaggtgctgcatggttgtcgtcagctcgtgccgtgaggtgtcggcttaagtgccataacgagcgcaacccctattgtcagttgccagcaggtaaagctggggactctgacgagactgccggcgcaagctgagaggaaggcggggatgacgtcaaatcagcacggcccttacgtccggggcgacacacgtgttacaatggcaggcacagcgggaagccacccggcgacggggagcggaacccgaaagcctgtctcagttcggatcggagtctgcaactcgactccgtgaagctggattcgctagtaatcgcgcatcagccatggcgcggtgaatacgttcccgggccttgtacacaccgcccgta

SEQ ID NO: 77 - DNA, 1357 bp, Collinsella sp.; identical to SEQ ID NO: 12
  modified_base 766: mod_base = OTHER; note = a, c, t, g, unknown or other
  source 1..1357: mol_type = genomic DNA

SEQ ID NO: 78 - DNA, 1432 bp, Phascolarctobacterium sp.
  source 1..1432: mol_type = genomic DNA
agagttgatctggctcagattgaacgctggcggcaggcttaatacatgcaagtcgaacggtaacagcaaaaaagcttgcttttttggctgacgagtggcggacgggtgagtaatacctaggaagctgcctaaacgagggggataacacctggaaacgggtgctaataccgcatgataccgcaaggtcaaaggttggtttaccaatcgcgtttagatgcgcctaggagggattagctagttggtggggtaacggctcaccaaggcgatgatcagtagccggtctgagaggatgaacggccacattgggactgagacacggcccagactcctacgggaggcagcagtggggaatcttccgcaatgggcgaaagcctgacggagcaatgccgcgtgagtgatgaagggattcgtcccgtaaagctctgttgtatatgacgaatgtgcagattgtgaataatgatttgtaatgacggtagtatacgaggaagccacggctaactacgtgccagcagccgcggtaatacgtaggtggcgagcgttgtccggaattattgggcgtaaagagcatgtaggcggttttttaagtctggagtgaaaatgcggggctcaaccccgtatggctctggatactggaagacttgagtgcaggagaggaaaggggaattcccagtgtagcggtgaaatgcgtagatattgggaggaacaccagtggcgaaggcgcctttctggactgtgtctgacgctgagatgcgaaagccagggtagcgaacgggattagataccccggtagtcctggccgtaaacgatgggtactaggtgtgggaggtatcgaccccttccgtgccggagttaacgcaataagtaccccgcctggggagtacgtccgcaaggatgaaactcaaaggaattgacgggggcccgcacaagcggtggagtatgtggtttaattcgacgcaacgcgaagaaccttaccaaggcttgacattgattgaaagacctagagataggtccctctcttcggagacaagaaaacaggtggtgcatggctgtcgtcagctcgtgtcgtgagatgttgggttaagtcccgcaacgagcgcaacccctatcctatgttaccagcgggtaatgccggggactcataggagactgccaaggacaacttggaggaaggcggggatgacgtcaagtcatcatgccccttatgtcttgggctacacacgtactacaatggtcggcaacagagggaagcaaagccgcgaggcagagcaaaccccagaaacccgatctcagttcggattgcaggctgcaactcgcctgcatgaagtcggaatcgctagtaatcgcaggtcagcatactgcggtgattactatcccgggcgttgtactcaccgcccgtcaggcggagttcgtacttcaaatgtgccacactggg

SEQ ID NO: 79 - DNA, 253 bp, Clostridium sp.
  source 1..253: mol_type = genomic DNA
tacgtaggtggcaagcgttgtccggatttactgggcgtaaagggagcgtaggcggatttttaagtgggatgtgaaatacccgggctcaacctgggtgctgcattccaaactggaaatctagagtgcaggaggggaaagtggaattcctagtgtagcggtgaaatgcgtagagattaggaagaacaccagtggcgaaggcgactttctggactgtaactgacgctgaggctcgaaagcgtggggagcaaacagg

SEQ ID NO: 80 - DNA, 253 bp, Clostridium sp.; identical to SEQ ID NO: 14
  source 1..253: mol_type = genomic DNA

SEQ ID NO: 81 - DNA, 1402 bp, Turicibacter sp.
  source 1..1402: mol_type = genomic DNA
agagtttgatcctggctcaggatgaacgctagcgataggcctaacacatgcaagtcgaggggcagcacatgagtagcaatacgatggtggcgaccggcgcacgggtgagtaacacgtatgcaacctacctttaacaggggaataacccgttgaaaaacggactaatactccataacacaggggtcccgcatgggaatatttgttaaagatttatcggttgaagatgggcatgcgttccattagctagttggtagggtaaaggcctaccaaggcgacgatgcgtagccgacctgagagggtgaacggccacactgggactgagacacggcccacactcctacgggaggcagcagtagggaatcttcggcaatgggcgaaagcctgaccgagcaacgccgcgtgaatgatgaaggccttcgggttgtaaaattctgttataagggaagaacgactttagtaggaaatggctagagtgtgacggtaccttatgagaaagccacggctaactacgtgccagcagccgcggtaatacgtaggtggcgagcgttatccggaattattgggcgtaaagagcgcgcaggtggttgattaagtctgatgtgaaagcccacggcttaaccgtggagggtcattggaaactggtcgacttgagtgcagaagagggaagtggaattccatgtgtagcggtgaaatgcgtagagatatggaggaacaccagtggcgaaggcggcttcctggtctgtaactgacactgaggcgcgaaagcgtggggagcaaacaggattagataccctggtagtccacgccgtaaacgatgagtgctaagtgttgggggtcgaacctcagtgctgaagttaacgcattaagcactccgcctggggagtacggtcgcaagactgaaactcaaaggaattgacggggacccgcacaagcggtggagcatgtggtttaattcgaagcaacgcgaagaaccttaccaggtcttgacataccattgaccgttctagagataggattttcccttcggggacaatggatacaggtggtgcatggttgtcgtcagctcgtgtcgtgagatgttgggttaggtcccgcaacgagcgcaacccctgtcgttagttgccagcattcagttggggactctaacgagactgccagtgacaaactggaggaaggtggggatgacgtcaaatcatcatgccccttatgacctgggctacacacgtgctacaatggttggtacaaagagaagcgaagcggtgacgtggagcaaacctcataaagccaatctcagttcggattgtaggctgcaactcgcctacatgaagttggaatcgctagtaatcgcgaatcagaatgtcgcggtgaatacgttcccgggtcttgtacacaccgcccgtca

SEQ ID NO: 82 - DNA, 1409 bp, Streptococcus sp.
  source 1..1409: mol_type = genomic DNA
tgcaagtagaacgctgaagactggtgcttgcaccggttggaagagttgcgaacgggtgagtaacgcgtaggtaacctgcctgatagcgggggataactattggaaacgatagctaataccgcataacagggaataacacatgttatttttttgaaaggggcaattgctccactatcagatggacctgcgttgtattagctagtaggtgaggtaacggctcacctaggcgacgatacatagccgacctgagagggtgatcggccacactgggactgagacacggcccagactcctacgggaggcagcagtagggaatcttcggcaatgggggcaaccctgaccgagcaacgccgcgtgagtgaagaaggttttcggatcgtaaagctctgttgtaagagaagaacgttgagtagagtggaaagttactcaagtgacggtatcttaccagaaagggacggctaactacgtgccagcagccgcggtaatacgtaggtcccgagcgttgtccggatttattgggcgtaaagcgagcgcaggcggtttaataagtctgaagttaaaggcagtggctcaaccattgttcgctttggaaactgttaaacttgagtgcagaaggggagagtggaattccatgtgtagcggtgaaatgcgtagatatatggaggaacaccggtggcgaaagcggctctctggtctgtaactgacgctgaggctcgaaagcgtgggtagcgaacaggattagataccctggtagtccacgccgtaaacgatgagtgctaggtgttgggtcctttccgggactcagtgccgacgctaacgcattaagcactccgcctggggagtacgaccgcaaggttgaaactcaaaggaattgacgggggcccgcacaagcggtggagcatgtggtttaattcgaagcaacgcgaagaaccttaccaggtcttgacatcccgatgctatccctagagatagggagttacttcggtacatcggtgacaggtggtgcatggttgtcgtcagctcgtgtcgtgagatgttgggttaagtcccgcaacgagcgcaacccctattgttagttgccatcattcagttgggcactctagcgagactgccggtaataaaccggaggaaggtggggatgacgtcaaatcatcatgccccttatgacctgggctacacacgtgctacaatggttggtacaacgagttgcgagtcggtgacggcaagctaatctcttaaagccaatctcagttcggattgtaggctgcaactcgcctacatgaagtcggaatcgctagtaatcgcggatcagcacgccgcggtgaatacgttcccgggccttgtacacaccgcccgtcacaccacgagagtttgtaacacccaaagtcggtgaggtaaccttcggagcc

SEQ ID NO: 83 - DNA, 1517 bp, Streptococcus sp.; identical to SEQ ID NO: 50
  source 1..1517: mol_type = genomic DNA

SEQ ID NO: 84 - DNA, 252 bp, Streptococcus sp.; identical to SEQ ID NO: 51
  source 1..252: mol_type = genomic DNA

SEQ ID NO: 85 - DNA, 1422 bp, Streptococcus sp.
  source 1..1422: mol_type = genomic DNA
agagtttgatcctggctcaggacgaacgctggcggcgtgcctaatacatgcaagtcgagcgagcggaactaacagatttacttcggtaatgacgttaggaaagcgagcggcggatgggtgagtaacacgtggggaacctgccccatagtctgggataccacttggaaacaggtgctaataccggataagaaagcagatcgcatgatcagcttttaaaaggcggcgtaagctgtcgctatgggatggccccgcggtgcattagctagttggtaaggtaaaggcttaccaaggcaatgatgcatagccgagttgagagactgatcggccacattgggactgagacacggcccaaactcctacgggaggcagcagtagggaatcttccacaatggacgcaagtctgatggagcaacgccgcgtgagtgaagaaggttttcggatcgtaaagctctgttgttggtgaagaaggatagaggtagtaactggcctttatttgacggtaatcaaccagaaagtcacggctaactacgtgccagcagccgcggtaatacgtaggtggcaagcgttgtccggatttattgggcgtaaagcgagcgcaggcggtttaataagtctgaagttaaaggcagtggcttaaccattgttcgctttggaaactgttagacttgagtgcagaaggggagagtggaattccatgtgtagcggtgaaatgcgtagatatatggaggaacaccggtggcgaaagcggctctctggtctgtaactgacgctgaggctcgaaagcgtggggagcaaacaggattagataccctggtagtccacgccgtaaacgatgagtgctaggtgttaggccctttccggggcttagtgccgcagctaacgcattaagcactccgcctggggagtacgaccgcaaggttgaaactcaaaggaattgacgggggcccgcacaagcggtggagcatgtggtttaattcgaagcaacgcgaagaaccttaccaggtcttgacatcccgatgctattcctagagataggaagtttcttcggaacatcggtgacaggtggtgcatggttgtcgtcagctcgtgtcgtgagatgttgggttaagtcccgcaacgagcgcaacccctattgttagttgccatcattaagttgggcactctagcgagactgccggtaataaaccggaggaaggtggggatgacgtcaagtcatcatgccccttatgacctgggctacacacgtgctacaatgggcagtacaacgagaagcgagcctgcgaaggcaagcgaatctctgaaagctgttctcagttcggactgcagtctgcaactcgactgcacgaagctggaatcgctagtaatcgcggatcagcacgccgcggtgaatacgttcccgggccttgcacacaccgcccgtca

SEQ ID NO: 86 - DNA, 1536 bp, Streptococcus sp.
  source 1..1536: mol_type = genomic DNA
agagtttgatcctggctcaggacgaacgctggcggcgtgcctaatacatgcaagtggaacgcacagttagtatgtagtttactacaacattacttgtgagtcgcgaacgggtgagtaacgcgtaggtaacctgccttgtagcgggggataactattggaaacgatagctaataccgcataacagttgataactcatgttattagcttgaaagatgcaacagcatcactacgagatggacctgcgttgtattagctagttggtgaggtaaaggctcaccaaggccacgatacatagccgacctgagagggtgatcggccacattgggactgagacacggcccaaactcctacgggaggcagcagtagggaatcttcggcaatgggggcaaccctgaccgagcaacgccgcgtgagtgaagaaggttttcggatcgtaaagctctgttgtaagagaagaacgttgatgagagtggaaaattcatcaagtgacggtatcttaccagaaagggacggctaactacgtgccagcagccgcggtaatacgtaggtcccgagcgttgtccggatttattgggcgtaaagcgagcgcaggcggtttcgtaagtctgaagttaaaggcagtggctcaaccattgttcgctttggaaactgcgagacttgagtgcagaaggggagagtggaattccatgtgtagcggtgaaatgcgtagatatatggaggaacaccggtggcgaaagcggctctctggtctgtaactgacgctgaggctcgaaagcgtggggagcaaacaggattagataccctggtagtccacgccgtaaacgatgagtgctaggtgttaggccctttccggggcttagtgccgcagctaacgcattaagcactccgcctggggagtacgaccgcaaggttgaaactcaaaggaattgacgggggcccgcacaagcggtggagcatgtggtttaattcgaagcaacgcgaagaaccttaccaggtcttgacatcccgatgcccgctctagagatagagttttacttttgtacatcggtgacaggtggtgcatggttgtcgtcagctcgtgtcgtgagatgttgggttaagtcccgcaacgagcgcaacccctattgttagttgccatcattgagttgggcactctagcgagactgccggtaataaaccggaggaaggtggggatgacgtcaaatcatcatgccccttatgacctgggctacacacgtgctacaatggctggtacaacgagtcgcaagccggtgacggcaagctaatctcttaaagccagtctcagttcggattgtaggctgcaactcgcctacatgaagtcggaatcgctagtaatcgcggatcagcacgccgcggtgaatacgttcccgggccttgtacacaccgcccgtcacaccacgagagtttgtaacacccgaagtcggtgaggtaaccttttaggagccagccgcctaaggtgggatagatgattggggtgaagtcgtaacaaggtagccgtatcggaaggtgcggctg

SEQ ID NO: 87 - DNA, 1393 bp, Streptococcus sp.; identical to SEQ ID NO: 32
  modified_base 1381: mod_base = OTHER; note = a, c, t, g, unknown or other
  source 1..1393: mol_type = genomic DNA

SEQ ID NO: 88 - DNA, 1510 bp, Streptococcus sp.
  source 1..1510: mol_type = genomic DNA
agagtttgatcctggctcaggacgaacgctggcggcgtgcctaatacatgcaagtagaacgctgaagaaaggagcttgcttcttttggatgagttgcgaacgggtgagtaacgcgtaggtaacctgccttgtagcgggggataactattggaaacgatagctaataccgcataacagcttttgacacatgttagaagcttgaaagatgcaattgcatcactacgagatggacctgcgttgtattagctagtaggtagggtaacggcctacctaggcgacgatacatagccgacctgagagggtgatcggccacactgggactgagacacggcccagactcctacgggaggcagcagtagggaatcttcggcaatgggggcaaccctgaccgagcaacgccgcgtgagtgaagaaggttttcggatcgtaaagctctgttgtaagagaagaacgtgtgtgagagtggaaagttcacacagtgacggtaacttaccagaaagggacggctaactacgtgccagcagccgcggtaatacgtaggtcccgagcgttgtccggatttattgggcgtaaagcgagcgcaggcggtttaataagtctgaagttaaaggcagtggcttaaccattgttcgctttggaaactgttaaacttgagtgcagaaggggagagtggaattccatgtgtagcggtgaaatgcgtagatatatggaggaacaccggtggcgaaagcggctctctggtctgtaactgacgctgaggctcgaaagcgtggggagcaaacaggattagataccctggtagtccacgccgtaaacgatgagtgctaggtgttaggccctttccggggcttagtgccgcagctaacgcattaagcactccgcctggggagtacgaccgcaaggttgaaactcaaaggaattgacgggggcccgcacaagcggtggagcatgtggtttaattcgaagcaacgcgaagaaccttaccaggtcttgacatcccagtgaccgctctagagatagagtttttcttcggaacactggtgacaggtggtgcatggttgtcgtcagctcgtgtcgtgagatgttgggttaagtcccgcaacgagcgcaacccttattgttagttgccatcattcagttgggcactctagcgagactgccggtaataaaccggaggaaggtggggatgacgtcaaatcatcatgccccttatgacctgggctacacacgtgctacaatggttggtacaacgagtcgcaagtcggtgacggcaagcaaatctcttaaagccaatctcagttcggattgtaggctgcaactcgcctacatgaagcaggaattgctagtaatggcaggtcagcatactgccgtgaatacgttcccgggccttgtacacaccgcccgtcacaccatgagagtctgtaacacccgaagtcggtagtctaactacggaggacgccgccgaaggtgggacagataattggggtgaagtcgtaacaaggtagccgta

SEQ ID NO: 89 - DNA, 1442 bp, Streptococcus sp.; identical to SEQ ID NO: 56
  source 1..1442: mol_type = genomic DNA

SEQ ID NO: 90 - DNA, 1397 bp, Anaerostipes sp.
  source 1..1397: mol_type = genomic DNA
ctacctgcagtcgacgaacaccttatttgattttcttcggaactgaagatttggtgattgagtggcggacgggtgagtaacgcgtgggtaacctgccctgtacagggggataacagtcagaaatgactgctaataccgcataagaccacagcaccgcatggtgcaggggtaaaaactccggtggtacaggatggacccgcgtctgattagctggttggtgaggtaacggctcaccaaggcgacgatcagtagccggcttgagaaagtgaacggccacattgggactgagacacggcccaaactcctacgggaggcagcagtggggaatattgcacaatgggggaaaccctgatgcagcgacgccgcgtgagtgaagaagtatctcggtatgtaaagctctatcagcagggaagaaaatgacggtacctgactaagaagccccggctaactacgtgccagcagccgcggtaatacgtagggggcaagcgttatccggaattactgggtgtaaagggtgcgtaggtggtatggcaagtcagaagtgaaaacccagggcttaactctgggactgcttttgaaactgtcagactggagtgcaggagaggtaagcggaattcctagtgtagcggtgaaatgcgtagatattaggaggaacatcagtggcgaaggcggcttactggactgaaactgacactgaggcacgaaagcgtggggagcaaacaggattagataccctggtagtccacgccgtaaacgatgaatactaggtgtcggggccgtagaggcttcggtgccgcagccaacgcagtaagtattccacctggggagtacgttcgcaagaatgaaactcaaaggaattgacggggacccgcacaagtagcggagcatgtggtttaattcgaagcaacgcgaagaaccttacctaagcttgacatccttttgaccgatgcctaatcgcatctttcccttcggggacagaagtgacaggtggtgcatggttgtcgtcagctcgtgtcgtgagatgttgggttaagtcccgcaacgagcgcaacccttgcctttagttgccatcattaagttgggcactctagagggactgccagggataacctggaggaaggtggggatgacgtcaaatcatcatgccccttatgcttagggctacacacgtgctacaatgggtggtacagagggcagcgaagtcgtgaggccaagctaatcccttaaagccattctcagttcggattgtaggctgaaacccgcctacatgaagctggagttactagtaatcgcagatcagaatgctgcggtgaatgcgttcccgggtcttgtacacaccgcccgtcacaccatgggagttgggggcgcccgaagccggctagctactttggaagcgt

SEQ ID NO: 91 - DNA, 1435 bp, Lachnoclostridium sp.
  source 1..1435: mol_type = genomic DNA
ggggggcttaacacatgcaagtcgaacgaagcgctttcgctttaatcttcggaggaaagaggaagtgactgagtggcggacgggtgagtaacgcgtgggtaacctgcctcatacagggggataacagttagaaatggctgctaataccgcataagcatacagcaccgcatggtgcagtgtgaaaaactccggtggtataagatggacccgcgtctgattaggtagttggtggggtaacggcctaccaagccgacgatcagtagccgacctgagagggtgaccggccacattgggactgagacacggcccaaactcctacgggaggcagcagtggggaatattgcacaatgggggaaaccctgatgcagcgacgccgcgtgaaggaagaagtatttcggtatgtaaacttctatcagcagggaagaaaatgacggtacctgactaagaagccccggctaactacgtgccagcagccgcggtaatacgtagggggcaagcgttatccggatttactgggtgtaaagggagcgtagacggaagtgcaagtctgaagtgaaagcccggggctcaaccccgtgactgctttggaaactgtgcttctagagtgtcggagaggtaagcggaattcctagtgtagcggtgaaatgcgtagatattaggaggaacatcagtggcgaaggcggcttactgggcgataactgacgttgaggctcgaaagcgtggggagcaaacaggattagataccctggtagtccacgccgtaaacgatgaatactaggtgtcgggaagcacagcttttcggtgccgccgcaaacgcattaagtattccacctggggagtacgttcgcaagaatgaaactcaaaggaattgacggggacccgcacaagcggtggagcatgtggtttaattcgaagcaacgcgaagaaccttaccaagtcttgacatcccggtgaccggacagtaatgtgtccttttcttcggaacaccggtgacaggtggtgcatggttgtcgtcagctcgtgtcgtgagatgttgggttaagtcccgcaacgagcgcaacccttatccccagtagccagcggttcggccgggcactctgaggagactgccagggataacctggaggaaggtggggatgacgtcaaatcatcatgccccttatgacttgggctacacacgtgctacaatggcgtaaacaaagggaagcgagaccgtgaggtggagcaaatcccaaaaataacgtctcagttcggactgtagtctgcaacccgactacacgaagctggaatcgctagtaatcgcagatcagaatgctgcggtgaatacgttcccgggtcttgtacacaccgcccgtcacaccatgggagttggaaatgcccgaagtcagtgacccaaccgcaaggagggagctgccgaaggcaggttcgataactg

SEQ ID NO: 92 - DNA, 1493 bp, Roseburia sp.
  source 1..1493: mol_type = genomic DNA
agagtttgatcctggctcaggatgaacgctggcggcgtgcttaacacatgcaagtcgaacgaagcactttaacttgattttttcggaatgattgttcttgtgactgagtggcggacgggtgagtaacgcgtgggtaacctgcctcatacagggggataacagttagaaatgactgctaataccgcataagcgcacggtatcgcatgatacagtgtgaaaaactccggtggtatgagatggacccgcgtctgattagctagttggcggggtaacggcccaccaaggcgacgatcagtagccgacctgagagggtgaccggccacattgggactgagacacggcccaaactcctacgggaggcagcagtggggaatattgcacaatgggcgaaagcctgatgcagcgacgccgcgtgaacgaaaaagtatttcggtatgtaaagttctatcagcagggaagataatgacggtacctgactaagaagcaccggctaaatacgtgccagcagccgcggtaatacgtatggtgcaagcgttatccggatttactgggtgtaaagggagcgcaggcggtacggcaagtctgatgtgaaagcccggggctcaaccccggtactgcattggaaactgtcgaactagagtgtcggaggggtaagcggaattcctagtgtagcggtgaaatgcgtagatattaggaggaacaccagtggcgaaggcggcttactggacgacaactgacgctgaggcgcgaaagcgtggggagcaaacaggattagataccctggtagtccacgctgtaaacgatgaatactaggtgtgggaggactgaccccttccgtgccgcagttaacacaataagtattccacctggggagtacggccgcaaggctgaaactcaaaggaattgacgggggcccgcacaagcagtggattatgtggtttaattcgacgcaacgcgaagaaccttaccaggacttgacatccaactaacgaagtagagatacattaggtgcccttcggggaaagttgagacaggtggtgcatggttgtcgtcagctcgtgtcgtgagatgttgggttaagtcccgcaacgagcgcaacccctattgttagttgctacgcaagagcactctagcgagactgccgttgacaaaacggaggaaggcggggacgacgtcaaatcatcatgccccttatgtcctgggctacacacgtaatacaatggccgtcaacaaagggaagcaaagccgcgaggtggagcaaatccccaaaaacggtctcagttcggattgcaggctgcaactcgcctgcatgaagctggaattgctagtaatcgtggatcagcatgccacggtgaatacgttcccgggccttgtacacaccgcccgtcacaccatgagagtcgggaacacccgaagtccgtagtctaaccgcaaggagggcgcggccgaaggtgggtccggtaattggggtgaagtcgtaacaaggtaaccgt

SEQ ID NO: 93 - DNA, 1289 bp, Fusobacterium sp.
  source 1..1289: mol_type = genomic DNA
agtggcgaacgggtgagtaacgcgtgaggaacctgcctttcagtgggggacaacagttggaaacgactgctaataccgcatgatactttttggaggcatctctgaaaagtcaaagctttatgtgctgaaagatggtctcgcgtctgattagctagttggtgaggtaacggctcaccaaggcgacgatcagtagccggtctgagaggatgaacggccacattgggactgagatacggcccagactcctacgggaggcagcagtggggaatattgggcaatgggggaaaccctgacccagcaacgccgcgtgaaggaagaaggccttcgggttgtaaacttcttttaccagggacgaagaacgtgacggtacctggagaaaaagcaacggctaactacgtgccagcagccgcggtaatacgtaggttgcaagcgttatccggatttattgggcgtaaagcgcgtctaggcggtttggtaagtctgatgtgaaaatgcggggctcaactccgtattgcgttggaaactgctaaactagagtactggagaggtaggcggaactacaagtgtagaggtgaaattcgtagatatttgtaggaatgccgatggggaagccagcctactggacagatactgacgctaaagcgcgaaagcgtggggagcaaacaggattagataccctggtagtccacgctgtaaacgatgagtactaggtgtcggaggttacccccttcggtgccgcagctaacgcattaagtactccgcctggggagtacgcacgcaagtgtggaactcaaaggaattgacggggacccgcacaagtagcggagcatgtggtttaattcgaagcaacgcgaagaaccttacctaggcttgacatccttctgaccgaggactaatctcctctttccctccggggacagaagtgacaggtggtgcatggttgtcgtcagctcgtgtcgtgagatgttgggttaagtcccgcaacgagcgcaacccttgtctttagttgccatcatttagttgggcactctggagagactgccagggataacctggaggaaggtggggatgacgtcaaatcatcatgccccttatgcctagggctacacacgtgctacaatgggtggtacagagggcagctaagccgtgaggtggagcaaatcccttaaagccattctcagttcggattgtaggctgaaactcgcctacatgaagctggagttactagtaatcgcagatcagaatgctgcggtgaatgcgttcccgggtcttgtacacaccgcccgtca

SEQ ID NO: 94 - DNA, 1366 bp, Fusobacterium sp.; identical to SEQ ID NO: 37
  source 1..1366: mol_type = genomic DNA

SEQ ID NO: 95 - DNA, 1361 bp, Fusobacterium sp.; identical to SEQ ID NO: 70
  source 1..1361: mol_type = genomic DNA

SEQ ID NO: 96 - DNA, 1415 bp, Fusobacterium sp.
  source 1..1415: mol_type = genomic DNA
aatgcttaacacatgcaagtctacttgatccttcgggtgatggtggcggacgggtgagtaacgcgtaaagaacttgccttgcagtctgggacaacgtctggaaacggacgctaataccggatattatgcgagagtcgcatggctctttcatgaaagctatatgcgctgcaggagagctttgcgtcccattagttagttggtgaggtaacggctcaccaagaccgcgatgggtagccggcctgagagggtgaacggccacaaggggactgagacacggcccttactcctacgggaggcagcagtggggaatattggacaatggaccaaaagtctgatccagcaattctgtgtgcacgatgacggtcttaggattgtaaagtgctttcaatcgggaaaaagaaagtgatggtaccgatagaagaagcgacggctaaatacgtgccagcagccgcggtaatacgtatgtcgcaagcgttatccggatttattgggcgtaaagcgcgtctaggcggtctggtaagtctgatgtggaaatgcggggctcaactccgtattgcgttggaaactgccagactagagtactggagaggtgggcggaactacaagtgtagaggtgaaattcgtagatatttgtaggaatgccgatagagaagtcagctcactggacagatactgacgctgaagcgcgaaagcatggggagcaaacaggattagataccctggtagtccatgccgtaaacgatgattactaagcgtcgggggtcgaacctcggcactcaagctaacgcgataagtaatccgcctggggagtacgtacgcaagtatgaaactcaaaggaattgacggggacccgcacaagtggtggagcatgtggtttaattggacgcaacgcgaggaactttaccagcgtgtgacatcctaggaatgagaaagagatttttcagtgctccttcgggagaacccagagacaggtggtgcatggctgtggtcagctcgtgtcgtgagatgttgggttaagtcccgcaacgagcgcaacccctattgtatgttgccatcattaagttgggcaatcatgcgatgctgcctgcgacgagcaggaggaaggtggggatgaggtcaagtcatcatgcccgttatatgctgggctacacacgtgctacaatgggcagtacagagagaagcaaatatgcgaggaggagcaaatgtcagaaagctgttcgtagttcggattgtactctgcaactggagtacatgaagttggaatcagtagtaatcgcaaatcagcaatgttgcggtgaatacgttctcgggtctggtacacaccgcccgtcacaccacgagagttgattgcacctgaagtagcaggcctaaccgtaaggaagggtggtccgagggtgtggttagcgattggggtg

SEQ ID NO: 97 - DNA, 1395 bp, unidentified
  misc_feature 1..1395: note = source = /note="Description of Unknown: Lachnospiraceae sequence"
  source 1..1395: mol_type = genomic DNA
agagtttgatcctggctcaggatgaacgctggcggcgtgcttaacacatgcaagtcgagcgaagcgcttttacggatttcttcggattgaagtgattgtgactgagcggcggacgggtgagtaacgcgtgggtaacctgcctcatacagggggataacagttagaaatgactgctaataccgcataagcgcacagtaccgcatgggtacggtgtgaaaaactccggtggtatgagatggacccgcgtctgattaggtagttggtggggtaacggcctaccaagccaacgatcagtagccgacctgagagggcgaccggccacattgggactgagacacggcccaaactcctacgggaggcagcagtggggaatattgcacaatgggggaaaccctgatgcagcgacgccgcgtgaaggatgaagtatttcggtatgtaaacttctatcagcagggaagaaaataacggtacctgagtaagaagccccggctaactacgtgccagcagccgcggtaatacgtagggggcaagcgttatccggatttactgggtgtaaagggagcgtagacggaagtgcaagtctgatgtgaaaacccgaggctcaaccacgggactgcattggaaactgtgcttctagagtgccggagaggtaagcggaattcctagtgtagcggtgaaatgcgtagatattaggaggaacaccagtggcgaaggcggcttactggacggtaactgacgttgaggctcgaaagcgtggggagcaaacaggattagataccctggtagtccacgccgtaaacgatgacttactagggtgtcgggcagcaaagctgttcggttgccgcagccatcgcaataagtagtccacctgggggagtacgttcgcaagaatgaaactcaaaggaattgacggggacccgcacaagcggtggagcatgtggtttaattcgaagcaacgcgaagaaccttacctgctcttgacatccctctgaccggcaagtaatgttgcctttccttcgggacagaggagacaggtggtgcatggttgtcgtcagctcgtgtcgtgagatgttgggttaagtcccgcaacgagcgcaacccctatcttcagtagccagcatttaaggtgggcactcaggagagactgccagggataacctggaggaaggtggggatgacgtcaaatcatcatgccccttatgagcagggctacacacgtgctacaatggcgtaaacaaagggaagcgaaagggtgacctggagcaaatctcagaaataacgtctcagttcggattgtagtctgcaactcgactacatgaagctggaatcgctagtaatcgcgaatcagcatgtcgcggtgaatacgttcccgggtcttgtactcaccgcccgtca

SEQ ID NO: 98 - DNA, 1388 bp, unidentified
  misc_feature 1..1388: note = source = /note="Description of Unknown: Peptostreptococcaceae sequence"
  source 1..1388: mol_type = genomic DNA
agagtttgatcctggctcaggatgaacgctggcggcgtgcctaacacatgcaagttgagcgatttacttcggtaaagagcggcggacgggtgagtaacgcgtgggtaacctaccctgtacacacggataacataccgaaaggtatgctaatacgggataatatatttgagaggcatctcttgaatatcaaaggtgagccagtacaggatggacccgcgtctgattagctagttggtaaggtaacggcttaccaaggcgacgatcagtagccgacctgagagggtgatcggccacattggaactgagacacggtccaaactcctacgggaggcagcagtggggaatattgcacaatgggcgaaagcctgatgcagcaacgccgcgtgagtgatgaaggccttcgggtcgtaaaactctgtcctcaaggaagataatgacggtacttgaggaggaagccccggctaactacgtgccagcagccgcggtaatacgtagggggctagcgttatccggatttactgggcgtaaagggtgcgtaggcggtctttcaagtcaggagtgaaaggctacggctcaaccgtagtaagctcttgaaactgggagacttgagtgcaggagaggagagtggaattcctagtgtagcggtgaaatgcgtagatattaggaggaacaccagttgcgaaggcggctctctggactgtaactgacgctgaggcacgaaagcgtggggagcaaacaggattagataccctggtagtccacgctgtaaacgatgagtactaggtgtcgggggttacccccttcggtgccgcagctaacgcattaagtactccgcctgggaagtacgctcgcaagagtgaaactcaaaggaattgacggggacccgcacaagtagcggagcatgtggtttaattcgaagcaacgcgaagaaccttacctaagcttgacatcccaatgacatctccttaatcggagagttcccttcggggacattggtgacaggtggtgcatggttgtcgtcagctcgtgtcgtgagatgttgggttaagtcccgcaacgagcgcaacccttgtctttagttgccatcattaagttgggcactctagagagactgccagggataacctggaggaaggtggggatgacgtcaaatcatcatgccccttatgcttagggctacacacgtgctgattatgctaaggaaataggatttactggacaattcttaatagagcctaagccaaaagagcctactaaacatcaatatgattttgatactgctactgttttaggatttttaagaaagtataatctggataaatacttcaaagtgaatatagaagcaaaccatgcaacacttgcaggacatactttccaacatgaattaa

SEQ ID NO: 99 - DNA, 1457 bp, unidentified
  misc_feature 1..1457: note = source = /note="Description of Unknown: Lachnospiraceae sequence"
  source 1..1457: mol_type = genomic DNA
cgctggcggcgtgcttaacacatgcaagtcgaacgaagcgatttggaggaagttttcggatgaaatctgaattgactgagtggcggacgggtgagtaacgcgtgggtaacctgcctcacacagggggacaacagttagaaatggctgctaataccgcataagcgcacagcttcgcatgaagcagtgtgaaaaactccggtggtgtgagatggacccgcgtctgattaggtagttggtggggtaacggcctaccaagccgacgatcagtagccgacctgagagggtgaccggccacattgggactgagacacggcccaaactcctacgggaggcagcagtggggaatattgcacaatgggggaaaccctgatgcagcgacgccgcgtgagtgaagaagtatttcggtatgtaaagctctatcagcagggaagaaaatgacggtacctgactaagaagccccggctaactacgtgccagcagccgcggtaatacgtagggggcaagcgttatccggatttactgggtgtaaagggagcgtagacggcttggcaagtctgaagtgaaagcccggggctcaaccccgggactgctttggaaactgtcaggctagagtgctggagaggtaagtggaattcctagtgtagcggtgaaatgcatagatattaggaggaacaccagtggcgaaggcggcttactggacagtaactgacgttgaggctcgaaagcgtggggagcaaacaggattagataccctggtagtccacgccgtaaacgatgaatactaggtgttggggagcaaagctcttcggtgccgtcgcaaacgcaataagtattccacctgggaagtacgttcgcaagaatgaaactcaaaggaattgacggggacccgcacaagcggtggagcatgtggtttaattcgaagcaacgcgaagaaccttaccaagtcttgacatcccattgaaaagcccgtaacggggttccctcttcggagcaatggagacaggtggtgcatggttgtcgtcagctcgtgtcgtgagatgttgggttaagtcccgcaacgagcgcaacccttatcctaagtagccagcaggtagagctgggcactcttgggagactgccagggacaacctggaggaaggtggggatgacgtcaaatcatcatgccccttatgatttgggctacacacgtgctacaatggcgtaaacaaagggaagcgaagctgtgaagctaagcaaatctcaaaaataacgtctcagttcggattgtagtctgcaactcgactacatgaagctggaatcgctagtaatcgcggatcagaatgccgcggtgaacacgttcccgggtcttgtacacaccgcccgtcacaccatgggagtcagtaacgcccgaagccagtgacctaaccgcaaggaaggagctgtcgaaggcgggaccgataactggggtgaagtcgtaa